European Patent Application EP 4 180 540 A1, published May 17, 2023. Title: METHOD FOR ASSESSING PROGNOSIS OR RISK STRATIFICATION OF LIVER CANCER BY USING CPG METHYLATION VARIATION IN GENE. Applicant: Lepidyne Co., Ltd. The sequence listing filed with the application follows.

SEQUENCE LISTING (44 sequences)

SEQ ID NO: 1 - DNA, 552 bp, Homo sapiens
  source 1..552: mol_type = genomic DNA
tcgccctctggctcggcacggaggggggcgctcagcctttctggggcaaatttagtaatatgggacccgagccctcgacccgaaatacgcccgaggcatttatcctaaaaaacgacaaggtccgggcgcccagcagaacggcccggctcgaccgcgcgcagcttgcaggcaggggggtgtgcaggtcaccgcgccaccccggcgagcagagccgcggagggcgccacgtcggtgcgctggccccgcccgagcggggcgggaccttcctgtacccccggaagcccccgcgggcagctggggaggaaaccgcggccacgcgctcggggggcccggctcgggaagggcagtgcgcgcgcatgcgttggggcggggcgcctgggacctgcgggccccaggcccagcgcgccgccagccggagtgcccggcgcccgtcgaaaggcccctgcgccggttcaggacccgcacccagctacgctgcggagccccagctcgcagcaccctcccacccaccgctcctggctgcttttctcctgagtctgcggggcggggtcg

SEQ ID NO: 2 - DNA, 1074 bp, Homo sapiens
  source 1..1074: mol_type = genomic DNA
gcggcagcaggtgccggcagcgcggggaccgatcgatggagagaaggcgggcaagacgccgggaagcgcattcctcctcaaccgagtgccacaaccgccctcccgaagtgccccggggcttcgagcatcacctcgcggtaatccgggagggtggagggatgcggctggacccgggcgttgcgtgctccacacagcgcccagcccgtgccagccccgcgcccacctctccacgacgctcgtgccgggatcagcgcgaagccccttccagtccccgaagccctcgcccgcgcccgttctcccccagctcgccccctccagcccgctgcgccttgccgcagcatctccgggcactctgaggctgccgccgggacagggtcggagcgccgcagaacccaccgaaacttcccaggggggcaattcaaaattcgccggacgcgtcgccgccgcgcgcccctcggctcattcccttccgcgcgcccgcagccccaggctctccctctctcaggaccccccagcgccctgcgcggcgagaataggcccccaggtgcctcccggccccgggggctgccgtcgcacgtccgctcccgcaggggtcctcactccgccaatcgccgcggccgcgcgccctcgcgcacactcaccagcccgagccggggcggccatcttagcgctcaccccggccccccgccccccggttcggcggccgcgacgacccggtgcggcggctacgacagccgtgacgcgcagcaggccccgccccctcccacagccccacccctgcgccggctcttcgcgggcaccgagaacctgccggtggccgccttccgcgcctcgtgggggggtcggggccacggacggtccccggcgccgcaagtgggtctgcgcgaacaacaagcactgcctccccgggcgggcttcgcacctgtagtgccgtcgggacacgggagggtaaacccagcgtgtcctgtgtgcctgtgagccgcagaatcatccacggacgtcgttagtccttcctggaatttctgcgatttacacaacgtcgaattgtttggcagaaacgcgtggcaaactccg

SEQ ID NO: 3 - DNA, 5293 bp, Homo sapiens
  source 1..5293: mol_type = genomic DNA
acgcgccgagtttaagccctttctatttccctttaacgcttccgcaaatgccaagagaaatcgtaccaccgcagtgatatcattatttacatttaatttttaaaaattaaaactcaacagccacgcccattaagatgcagcgatgggcagccccggccacagaggctgcgggaggctggaggggttttgtcagccgcagtcacagccccgcggagctggcggcatttcagggcaggagacgggtcccccgagcccccggctgggcgctgcgggccttgcccagggggcctccggctccctgaccccgcgtgacccacgggaggccccgccgctccgcgggcggaattatttcggatttctctttgcggtcctagttcggaagaaactgctttccaccgcgggaagatctggcgggatggtgaccgaagggcctccgtgcagcggatcagacccggttccaccggctgagcccagggcgggcctatgggatccgctgatgcgcagagggactttggaaataatcagagcgaagccctcggccaagcgggaacgggtgcccggtggcaacgagtacgtggccccaaagcgggaaaacggaagaagaaaaacctcccgcggggactcgaggcgggtacgcggctcacccgccctttcgggaacccccaagcgcgtccgaatccgccccgaggcgaggcgggccgggccgtacctgctgctccgtccccggctccgtcccgggctcctggcggctgtcgctgcggttccttcccgcgggccgggccccttccctgcgccttcgccgcctcctcgcgcctgcccggggcccgcagcctccgcaccgggaacccggaggacccgaggcgggcgcaggggcgaagccggggccggggaggggccgcctcgctccgggttcgagacggaagaaacacgcggcgcaggctccggagcgacggctccgacggggacccgttaaataatttattgatgatacaaagcgactcgcgcccacccggggccgcccccggattctgcaaaaatagattcgcccccaccccgcgggtcctcacaaggcgtcccccgcgccgccgccgcacgggctgaccagcgccaagttcgagggtttgtgcttcttgagcagccgcgtgatcttctcgtcgtccgagttggggtccaggggccggttgtattcgtcgtcgtcctccgcgtccgagccgcccaccttcagcttctcggcgtccgagtcctgcttcttcttggccgacgccatctccaccgcgtgccgcttgcgccacttggtccggcggttctggaaccagacctgggagtggacggggcggtcaggcggccgcggggcccggggctggcgctggggccgttcgcaggacgcgggcccccggctctgctctcccgagccccgccgcgctcaccttcacctggctctcggtcatgcccagcgagtaggcgagacgcgcgcgctccgggcccgccaggtacttggtctgctcgaaggttttctccagcgcgaagatctgctggcccgagaaggtcgggcgcgagtgcttcttcttcccgtccttgtccaggacgccgccggccggggctgcaagggaggggaagggagggaggtcagcggccggcggggtccccctccgcgcccacccgccccgcaccccccgcgcgggccactcacccgggccagccagacgcgggtccctccagggcgcgccctgcaccacgccgggccagaagatgggcgggcgccccggcagctcggccaggggcttggggtagccgcgcgccacagcggccgcgggcccgaagtaaacgccggcggacgacgcgagcccgttgagccggggcagcccccccaggaggcccccgcccgccgcgcccacgggccggcccaggatgtcgctgatgccgtgcggggtcccgagcgggagctgcgcgcccaggccccccagcgcgggcgccttgaagccggccggaccctgcagcgcgtaggggaacagcgacgtcttcatctcggccatgttgtgcagcgcggccagcggggcactgctcagcacgaacgcgcccgggcggttagtgtccatgggcgccgccgccgccggcccgggctcccatccgggccccgccgccgccgcccctgcccgccggcccgggaagtttgcgcgcggcccgggcgggcgtcggctgcagcgcggggcgcggggcgcggggggcgggcgggcggctccggcgcggggcgggcgggcgggcggcggcggcggcggctccggggccggtcggagcggcgccgcgcgggacggacgcgctgataacgggggctccccggggcgcggcgcgcgcgctgattggctgcggaccccgcggtccggccattggccggcgccccccccccgcccgcgcgcccccgccggccgcgcactccatgaagggcccattagcgcggcaggtgcctcccgggctgtaaattcgccccgatttatctccccggggacgaaataaatccagcttggatgggagtgtagttaggcaaaggttttcatgcgaaatcaggaaaaaatacgagaacgtattttattaacggaaagaatgcagatttgaggacccgcccgcgcgctcggagcgccccactcggggaagagtcccggcccgcgtcccagtcgcgactgctccgccgcccgtggctggggtgggtgtgagcggcagcggacgccggcggggaacgcgctccgggcaggtcggggccacaggagggcggaggacgcgggcctcgagtccacggaatccacgggcctcacggccgggcgaggctcgcacggagctgcctctggtttcgccgacacgcggccggcgcggtggaggagtgaggcaggcgggagcggggcggggaggcgggtcccgggaccacacgcgcggctcggcacttccccgtcatcggcctccaggtctcccgctgggggtcccccaggatgtgacctgggcccacgacttcgcccacgggccgcctctcgcgaatccccggccgggagaacagagaccaggacggcctcagcgcggaagccctgtccagggcccgaacgtgggtgcgggctgggggcgcagcggcagaaacgcggccttagacgcgcgcggggggccggtgtcccccccgcccccacggcaccgggagccgctcgctcatccatcccgcagaccgggcggtgagatgactccgagccccgcgcacggcggccgcgagcaaacgctccgacgtctgtggtgacgtctcgtattgatttagggacacggggcggctgtggctgtggcccacggctcgtggggagcccgagtctgtgcgcagggaacgccgctgcgtggcctctctcgggcctgtgccgcggaggaaggcggcgcccggggttcggggccggggtctcacgtccgccccctcgcccccctccagcgtccgttttcgttttgtgcaggtcgaggcggggacttggcgccgtcggccgctcctggatggcggcttggaaaagccacctgcggccaaactccggggcagtggtgcggccgccgggtgtgtgcgcgctcggggctgccccggcggcttccggctccactgaggtgcagccccgcgttcacggggggttcgcttcccccgtcgactccgcactcgattcgactgggattgggattcgattgggcgcggccgccccaccggtgatcggcccccgcggagcctggcccgggaacccccagcgcccgtccggccccgagacccgccccggcctgtcctgcgccccgctccctcggaggagacacgaggaagggccctcccgggtcgggttcgggcccctcccagcaccccaaggcgacggcgcccgcgcccaaggctcgggctctgagctgagacgcgggaactgcggggccggggggggcgggcagggggagttgggggcgggggctgctgtcgccctgggatcccccactctgcgcggccgggcagaccctgggcgggccgggaggggtgcgggtcgcccgaactgaggcccaggaggcgcgcgcgggcggaacggcgggaggaagccgcgctcgggacaggctctggctcttctcacagcctggaggggcggggcagggggcgtcgctagcgctgttttatggctgaggaaacatggacctggaggcgctgcgctgcggcccgataaaccctgggtctgtctgcgccccccggtcctccctgggctgccgagggaacgcgtggggtcgcgggtggggctggcgtgtcactggctgcggagcgcgcggctctccagggctcaggggcgcgggatgaggggccagggtgagttgggggcgcagaggagccgggtaagggggggtccctctcccacgttcttgtaagccgtggaagtcttggcgcgctccgcaggtgccgcgtcctacccggctccccggcctgcgccccacgcgctttcccgccctcctcctcgcggagctgcgcgtgggtccggtggcttcacctcctacgcttcccggcgcccactccgggccccgtcccctctccggcccccgcccgcaccttttctcctgcgtcccccggtgccgccctctcggaaaccaccgaggcaactccccctcctcccgggaaggtccgagcgcctccgaccgcgatgtctttgcctgggctccgccgcccggcggccccgctgcctggagaggtccgcgatgccacctcctggcccgcgagcagatgtcccgcgaggaaggctgccggcatcggcgccgacgctccgcgctggaaaaccgagagcgcggggtttggcagaggccattcaagtttgttttactcgttcagcctgtatttgtggggctcctaccgcgcccgggctgtccggggggtgcaccgtgaacgcagcgggctccggcccgggcgcgggcgggtcagagcagcaaacgcgctcccccggcacccccgcggcgtctgcaggggagcgggcgacggggaggacggcgggggtgtcggcccggaaggagagccggcctaggccccggtgtccccgcgctgggggctgaggggcgacgggggaactccacagagggaaggagcctgcgttcgccttcggccgcccaggccatagagttcacaaactctgatttatcactgaggtgacttgtcccgcgcagccctaggcgagttgccaagctgcccgccctgaccgcgcccccaggccgggggtctcctagcagttcccggcaaaggccctgcattgtcttttttcccgaagtgagcgcattcccg

SEQ ID NO: 4 - DNA, 2001 bp, Homo sapiens
  source 1..2001: mol_type = genomic DNA
gcctcaccctggaacagggagtccagcaggtcctggttgacacagccggggctggcgtggtggacaaggaagcctggaccacagcagatgcatgagtgcaggccccacagccccccagggggaggctggcccagctcccaaagccccggtgccaggggcagtgtgaccccgggcggcctcacctataagcacggcggctgcccggcgcagggggtcctgtggactccgcaggtagccctgggtctggctcaggaagttgggcacgtggcctgggtatcgctgaacctggggacaaaagggctagtggcaggacaggagggctgatcctgagtgcggaggaggctgcagagctgaatccaggggccggggttccaggggagcccccagggcaggtggcatggtcggagaccttggacttgccccaccagtagcctatctggtttggctgcagtagaaacggttgggggccccggtgaaccctggaacaagtgggctgctgatcatacccccttgcggtcaccttgcttcccctactgaccaggcggcagcagaggtggctcagggcctcggggctgtcatagtgggccacggtgaccaactcctccagcaggccccagcaaaaggcgtggtcacagcgggccagggtccactctgagctctgggataggggaagtgagccgggtcaggggtccaggaagtagaaaggcaaaaggtggggtgggaagagggggagcaagggcatcgggtgaggggcagaagagcccagggcaggagactggattgattctgctcaagggaagagcagtagtaacctggccgcccgtcacacctgccactgaggtccttgggatgggtgagtccctgacctgtaattgtcggaggggaggcacggtgggagtggtgagtgttggatggcataggggtgggatggtgtcgggggctgctgacctcagcagcgtccctgctggggtcatgcaggcgcagcagcagcggcacgagactctgcagcaccagcttccgcagggggccgcggagccccagccggagcccgccccggccccggcgcaccagagtcccaaggagcccgacggccgaggcgcggattgagtcccgtgtctgcgtgggagggcgcagtcagggcaggcggagacagagaggggctgcaagggtgggagggggcggccagcgcggagcgaggaagcggcgggtctagggaaggctgctgactcggtgtgatctggggacagggaacagggcctggagctggacctggttgggaagcctggagagcccctgcagggggtggggcttgaagggatggggtccggaaggaaaagtcgagcggggaggagcttggcgggacacggccctggaggggcggagctgggcgacagcaggcgggaggggcgggggcggtcaggagggaagaaatctgggacggagacactggggggacggggcctgggagggagaaactggaggggcggggcggagcctgggaggtcagggcctgggagggacagactgacagactggggggcggggcatgggaaggagaaactagaggggcgggcggggcctgggaggcggggcctgggagggagagactgtaggggcggggcggggcatgagagggagaaacaggaggggcggggcggggcctgggagggagactgggggcggggcctgggagggagagactggaagggcggggcggggcctgagagggcggggcctgggcgggagagacgggggcggggcctgggagggagagactggaagggcgggggcggtgacagcggcaggggcgggacccggaggcggggcgtttgctcacgtcgtccagtagcggagggaggcgcggtcccagctccgcgctcaggagccgcacaggcgcccggggccgcagcaggagcctcctcagggcgcccagcgctgcacccacgagccgcgcgtcgccttcgcccagtgcgcccaggagcgccggcagcagcgtgctca

SEQ ID NO: 5 - DNA, 619 bp, Homo sapiens
  source 1..619: mol_type = genomic DNA
ccgtccgggactcggggggaggcgcgctgggtggtccggcagccgggggcgggcggtagcctgcaggcgtaattggcatgcacgccgttgtagctgagaccgcttaataaagcattacatatctcaccgcttccatatttcattacctcacgcggagcctgtgagagggccctaatgggagtcagctgtgtttttactttctgttgtcggccgggacgggtttctctgcggattctttgaaatgaaataatgtgatgcacgccgcgataagggccggcctgtaatgaggcccaggccgccgggcggctgctattgctccaggtgtcgcgtatttgggctgcgaggacaaggaggaggagggggcggcgccggaggatcgggggggagggggaagtcgcgaggggcagggggtgggagaaggcggagggaggaggcagggggcagggggcgggcggaagaggggaggaaggagggggcggcgggccgcggcaggccaggcgggagaagccggagacagagagaggacggggacagtggcggcctgcagagccctaggaacccgggttcaaatcctgcccgccagcgtgagagagcgtttgcccgcccaggcggtccaccg

SEQ ID NO: 6 - DNA, 2001 bp, Homo sapiens
  source 1..2001: mol_type = genomic DNA
ggctgccatttctcatggggttcgagccataagatgccaggtgtcagtcacctcagaagagagggttttgtttgtatttggtggggttcttccgggggtaccgaggctgaggactgatggatcgaggcgggtggatcacttgagttcggagttcgagaccagcctggccaacatggcgaaaccctgtctctactaaaaatacaaaaattagccaggtgaaaaattagccgggcatggtggtgcttgtctgtaatcccagctacatatgtaattccagctactcaggaagctgaggcaggagaattgcttgaacctgcggggcggaggttgcagtgagccgagatcgtgccactacactcccgtgagggagcagcctagggactaaggcccgctggctccgcgagatcagccaggcccgcatcatcccccaattacctgcagagggcgccgcagacacagagagggcgaggccgaggccgaggccatctaagcttctgggaagggggtcccaaagggaggccccgagctggagtccagggggcttggaaggaagaggtgaggacagcagaaaaggaaacgcaaattaaaagaagggaacgaaggctgggcgcggtggcttacgcctgtaagtccagcactttgggaggccgagtcgggaggatcgcttgaggtcaggagttcaagaccagcctggccaacatggtgaaacgccgtctctactaaaaatacaaaaaaattagccaggagtggtggcaggtgcctgtcatcccagctactccgcaggctgaggtgggaggatcgcttgagcccgggaggtgggggttgcagtgagccgagatcgcgccactgcactccaggctgggtgatagagtgagacccagtctcaaaaaaagagaaggaaaagagagaagggatggtggcggtgggggaggaaggcggttcttgtaatgatccgagaggagaccgcagcaccggttacgccctcgaacctcggcctcctcatctgcagaatggacgcagtccacaccgcgtgctgtggaagggttggagcgccggtttacatgacacagggctatcggctaagggggcgctgggaacgtggaaggtgctctatggtggggcgctgtagggtgctcttgggcagtagggttggagtcaaatctgggttgaagtccaacctaggttgaagtcctggctgccacctgacctctgcccctcagtttgctcatcagtaaaatggggttaaggaggctgcctcgcccagctccacggagccggaggtgatgaaggtcctggaagagcagaattcagaacccgagctttgggcggcggagcaggacagggcgcgggtgggcgcggcctccgggaggccagcacgagggggagcggcggggcccggacacacccagccagaaggaggaggccgaccccgcgccgactccgcagatgccgctcgggacttcgttgtccctccaggcgcccgccctggggtcctccatcacccgccgtcacctgggcgcggggaagctggcgggaggggaggcggggcttggcggcagcggcgggtgggggccggggagcgggggcaggggcgggcggacggagcgcggggctggggacccggggtcccagaagggggcgcggggacggggtccgaggagagggggccggggcggggcagggcggacagggctgggggcggaggtccgggggtgggtccggcggcgagtccgggtcggggcggacagagcagggggcgggggtccgggaggagggggccggggtccgggaggagggggcggggcccgggggcggggccggggtcggcgccctgcggggaggccggccacgtgacgcccgcggcccggcggggctgccaggcggcgagcgccgcggcggccccgggaggtggcggcgggcgcgagagcctgggccgcgcgggactgaccgtcggggccccgggacggcggccccggggcgcccatgccatggagaagctgg

SEQ ID NO: 7 - DNA, 3044 bp, Homo sapiens
  source 1..3044: mol_type = genomic DNA
gcgcgcgtgtggaaggctgggtggggtgcgcacacacgctcacttgtgtacgtacacacacacacacacacacacacacacaggcacacacacccgagctcagtcacccacattgcttgcccagggcgcctggaagagctggcgagcccgcccagctctgttcacccggccccgccccgccccctccgggagggctctccgggcggcgcccagccccgagcagagcaaaggacggcggcggccacctccgttctccggccgctggtttctcgtctttcctcgtcctttcattgaacccatctccgtgcttcgaaaatctgactctaacccgatctcttcgcgtctccgcctcttctttctagagtgagcgccaaaaagggcctgacagacagaagcctttggccccagcaccggcccagcccgtctctagacgattcttgctcctttcaccctcacagcctccagtggtcgcttcatcttcgcaccctcccggccaaccctaactctcctcgtctctcctcgcgctgtctcgcgtcctcccctcaggatccttccgcacattctcagcgtccagcgcggtttcccacaacttcctcacgccccgctcccctcgccctgtccccgccctcgacaccacctgcgttccccactcgctccaacctccctcccccgctatccccacttgtgggcctccagctctctgcccctttcctggcccccatccctgacaccccagggacccttcctccctcctcacgttctccctccttccaggatcccgccccgacacttcggggccctcccgctacgcgcactctttctcctcaggtcctgacacctgggcgccccctccctgtcacccaccttcagctccagccctgactctcgggcgccttgccacccttacgctccccgccccgccccggtccctcgggcgcccccactcgccgcctctacctccctacctgctacacctggcacccctgcccccacccctgctcatactcttcccccgcccccgacacctcgggcgccccctcacacgctcctattctccacacttccgtccccgaaaactcgggcgccctctcccttcacgctcagtctctcctccctccccgcccggccccggacccagcctggagatcgcgctcgggaggggcggctgccgcccgcggggcgcccgcggtgcccgggcctgggcagcgaggaggtgacgccgcccccgcgggatgagcccgggaggcggaggggcggaggaggtgctggcggcggcactgagcggcggcggcgcagggcgcgcgggccttccgcgccgactccatcgacccaaggggcggcggcggtggcggcggctgagcgaccctgggccgggcgcgtgatgaggaggggccggcgccagaccccgctgcacgtcggagctcgcctggatccgggcgttggcagccgaagggccctggccccgggactctccgccgctagcccccgtcatatcttctccgctttcgcttctccactctagccgggggtggggtgggtggggttggggtctccgcgggggtttccggccccgcggcccgctcccgggtgtgcctggaggagttctccctctgtggcgcgcgggagccctgtgatgcgtcagccggcgggacggatgagttgcttctccgggaaaccgtcctcgcttcctcacgaccctctcggctcccgcctgggtgcccctcgggccggcagtactccgcctccgggcgctcgaagcgagttccccgggggcttgttcgcaggcaccccttcccctccgaggcggcgcgcgcgctcccggccctgaccgcggccggacacactcgcgccccggtccgcctgtcgccctcccgcctgctccctccagtcaccccacccttagctgtccccgccaccttactccaccaccctcccccgcctctccgcgcactccgcgtcccggcctccagttcccctttcccttgaaccgctcacttcacagcccttcgcccccgggaagaagaaacatttcccgaagcgcactcctcagccctccttccccacgcgctcgccctcccctccccctgcttttcttgggggaggggggctgtcgccttggattgaaggccattgatttgtatgtatttgtcccagcgctggaggctgccccagccgccgcgccggtgccgccgctgccagtggagttgcctccccgcttccctagggtggttcggctccaccaaacatgtcggctcctgtcgggccccggggccgcctggctcccatcccggcggcctctcagccgcctctgcagcccgagatgcctgacctcagccacctcacggaggaggagaggaaaatcatcctggccgtcatggataggcagaagaaagaagaggagaaggagcagtccgtgctcaagtaaggacctggctccatattcccgcctctctccctgccctccgccccctcgcccactgccctgcggccgcctgcgcgccccagttcgccgccctccctcccgctggcggcgcccaggccacgagggctgcggccagcgccggccgcccgggctgttttaggggtgtctgagagcaggggtgtgtgtcggggagggagggcgccaaggccggctgaggtgagggtggcgagccttaggcggtgtgattttccttggcgcctttccggatttcctcgctggtcatcttggctccggggccccagcgggactggggctgaacccaggctctgtgcgtaccctctcctttcccgccgcgctgaggcagtgactggggcacagaatccaatatggccgtgcacaggtgctccctggacggacccgggcgaaggcgcgctggcaggggatgcggacgccaccctggtcccacgcctccgcggggcggctctaccagcaacgcgggacagagcagggctgcccacagtggctgcgagcagcgggcggcggcgcgggctaggggcctaagctctgtcgcggtcgggtgggtgtgcgtccgccgccatcttccagcccctccccctcggcg

SEQ ID NO: 8 - DNA, 801 bp, Homo sapiens
  source 1..801: mol_type = genomic DNA
ccgcggtgctacaggtttctggggccttcttcccggcagggccacgccggtttccaacgcggggggcatttttcggccttcccacggttcccgctgttcccacgaagacagtgtctgcggccaggcgctccgagagagatgcggccttccccgggccgggcctggccgcggcctgcccgtggtcccccgcagctcgggcccgcagcgcgaggccacagtccagggggagccggcaggcggcctcctccccgagccggaggagctgcgcggacgcagcggcttccaggccaccccaccccgcgccagcctgcacctgtgccgcctgggtgtcttccccgagactctggtactgtgaagggtccgggtcgcgcggggcgtcgtccggagcagggcggactcgggctttggcgcggcctttgccccggtttttggcgcgggaggactttcgaccccgacttcggccgctcatggtggcggcggaggcagcttcaaagacacgctgtgaccctgcggctcctgacgccagctctcggtcgggaccgagcgggtctctccacggcaaccgccgacgtcacgaacgtacaactgtaccgtcgcgagaggacgtgatgcgcccggtgattggcgccgccgctgcggctgcgcaggagacgacccccgcgggcgctcccacccccatctcgcgcggactcgctttaggtctcggcgagtttctctgatatgcgctcgcgggggtgctgccatttcatctcttccgcgcgggctcatcgtgctctcagggtctcgttgaacaaggcaacg

SEQ ID NO: 9 - DNA, 314 bp, Homo sapiens
  source 1..314: mol_type = genomic DNA
tcggccgcccgagggagtttcttttattcccagttcggctttcttttgcgaaggccgagatctgggcctgccaggggcctgcccgagtcctctatcgcgggtccacgtggccaccaatgacccgcggcgcccccgcgtgtccccgcagccactccgcggaagcagcggcgggagcgcaccaccttcacgcgttcacagctggacgtgctcgaggcgctcttcgccaagactcgctaccctgacatcttcatgcgggaggaggtggcgctcaagatcaacctgccggagtctagagtccaggtgcgcactccccg

SEQ ID NO: 10 - DNA, 2213 bp, Homo sapiens
  source 1..2213: mol_type = genomic DNA
ccggctttaaacgcctctccagccacctgtgaaccgcgaaggagccggctttcgcggcggggaccttgccaccagtaccctcgcgggccgaggtcgttctcccggtcggcttcccgcctcacccgaaaaggaattagagcatctacccaagacggtgactggcagggcagatcaaggtgtcctggtctcggccccagccccgcggtgcgccccgcccgcttaccttgaccgggtgcaggtagccatcgccgcgcagggcgcccaacccggcgtccgccggcgcctcggcgtcgtcctgcaggctgcgggtgagatgcgcgatgtaggtggtggccagcagcagcacgtccagcttggacagcttggtgtcgggcggcacggacggcagcgtgcgctgcagctccaggaaagcgtgccgcagggtctgcacccggctgcgctcccgcgccgcattcgccgccgccggccgcccgctcccggaacgcgagccgcccccagggcccgccggccccggcccggtccgcccgggacgcgagtcgcggatggcggcggccaggggcgcgggctcggcgctggcgctgagggggctgcccgctgggcggccgcggtccatggcagcttcccgcgccgcgcgcgctgcaaaggaccgaaggtgcggtgaggccggggggcggtcgggcttaacccgagaggcgcagccccctggttctccccgtgcgcccaccagcagcccaacggggctaagggcgctctcaagcgagctcgttttgcctgggacgcgatttgcttccggacgtctggggagagttgcggaactccggagttcttgggcttcctagaaggataagaagaggcgcagtgccggctttgcttttcaggggcaaattaagcaaaaggtctactctacccgggaagaaagatctcggaagcacagctcaggatcagcactcgttcgcgcttgggtgactttatccaacccggcacgcacgagaggtggcgcggctccttctcgccgacgccgcggaaaaccacggctcaccagccgccctcggcctttcacgccaggggggatttctgcccgaggagcgggggacccttagcctcacctcggggtacggcacccgccaccgttccgagcccgagagctgcgcagtacgcgtctgacgggcccctcacctttcctggagcggctgagtggagctccgctccgtcgtgagggcgggcgaggggcgtggagcagggcctgtgtggccagggccgcgctggtcactccatcctcgtccggccgatgcccaagtcgacggctgtttccaacctccgctggctgtgacttttatgcgggcgccccgcggccaggcgtgtgtgctccgaccggctaaggcaggtcgggcggaggacctggcccaccggagaggctacgccgggggctgaggcggcttagagggtcattaatcaaaccctccggcggggcgggctcgggggcggggcgtcctcctggccccgcccctcggctcactgcctcacgctgctttccccgaggcgcctcgctgagggcggcgtgtggagagtttggggtgtctgccgccggctgcggtggggccgggctggaggccgcgggtgaggcctgtggttaacctcgcgctgccgaggtcttacctcctcgagtccagtctgattccaggccgcttccaggccggtgcccagctgaggcgggaacgctgcagtttggttgagcgtgacttttaggctctgtgaggaaaagtcgagcgcgccacatcgaggcgctagccgtttattctaccacaaggtaaaagattcatgctgtcctagttaccctaaagctgggagatacactgcacttcctaccagaccccgaatgctctcagtgtctgtaattctttaagaagttcctagagcagacagcccttggatcgtgggcacttctccccggggacggggaccctgctgaccgcctccgctgcccccgcgggggccaccgctctttaattatttgggcgaaacattcttttctggttttgcacttgtggactcacgggaagcgtgacttgcagcgaggcaggacccgatcccaggcttctttagaaagcggacgctgcgccccaaggcctgttcagagccgccccaggaagccgtgggtccccgaccgccccaaaccgcagcggtttctgcaggtcctggacccgtcgccttcg

SEQ ID NO: 11 - DNA, 714 bp, Homo sapiens
  source 1..714: mol_type = genomic DNA
gcggacgcagtcacgagtccagggcgaagcaggcagggaggcaggtgggcctcggtccgccgcaagctcacacttaggaggaccacgggccgcatgctgtcgtcgtcaaggcaacgacctcactctgtccccaaccataggcacaaagtcttgggagacagatacggcccaggtcagaatgcgttcacggcaggcaccaacacctgtgaaggccaagggctagagagcaattagctgggtgagaggcaccacctcccagctcgtaaggcgcccagtacctggagcctgggaacctgcaccgctccaactacccctgggcgaaggcgttggccgcggagctgcaagggggggcggtttctcacccgccccgagagcgccaggcctcccttcttctgattggccgagccgagtcgtcacgagccatgattggctcagggccaaccaccccgccccttcacctagggctcggcccaggttctgctccctgacacgcagaggccctgcgtccccacacgccttggttctcgtcaggaggcgcctttctgccttccccagcgggaggaggcgattgtgatgcccacgcgaagggtaaaggtggcggttatgtaggactgcgaagactatgcaaaatgcgatacggtttccctcatagcatcgccgctggggcaggggcgggcgccgggcgccctgagtcgcgtaggcgcggcctgaccg

SEQ ID NO: 12 - DNA, 8078 bp, Homo sapiens
  source 1..8078: mol_type = genomic DNA
gcgggcaggcccaagctgcgatgtggagaattcgatgtccgagcgacctcctcggaggagtgggtcgagttaaatataaccgcgcgaatggaatggcgctaaaaataaggcagcagctggcctgtccacagccctgtcccgggaggggcgggggccccagtggtcttgggcaggaaggccgcgtccggcccaggggcgagaaggctgcggcgtccgcagccagggctggaaggcctgggaggccgcgctctgtgggccccggggcctccattcgggctgggtcgcgggcctggacggggactgtccagaggcatccgaaagccaggccaacttgcctggacgtaacaagacggaagggctgggcgctgaggtcctgccagcccggccgccagagggagctgagcgccagaggaggacaagccgaacccttcaggaggccgggcgtctccggagaccgaagcgccggaggacccgaggaggtctgccccgcgcgctgctctggagactcccggggcgggtggcgctcggcctttccgctcccttccttcccacaagtcccttcccgcgcgcgccccacggccctgcccgccctcccgcgtcagcgccccaaccgtcaagccagcaattgaaacgtttccaaaacggtctatttatttgctcccaataaatcgatcggcggtgattaaagaatcgatgtggcctgggtgggcgagtcgcttgaggggagggattgggggctttcgcccggcgcctgcagggaggccgagggcgggcgcgggcctgagggaggcgtgtcccgcccgggccacacccgaggacccgacacctgggctggcaggccccggcaggcagcgttccctccggcggagaggggcgcgcgcccgccgcctgctttcctcggcccctctcgcctttctcgcgcgccggggaggctgtggccgccagtggctgcggagctgctcagaggcttttgttgctcctcggccggctgaatggggattttgtaaagcgggacagataaaaatgagcagcatcatattgtttgacagaatgatctcgcatgatgaagtgtcggctccgaagggggtgaaaatggtgaattcctaaaaacccagccctgggctcctcctcgagctgccggtagcctggagggacccagcggacagccgggcctggccgcatcgctccaaacggtgtcagaaagactccggctttcaatgccaagtcatttttaagccccgatcctgtccaggacctttctcctcgtggatgaaaagaacaattttcgagagaaaggctcgtttttattaaatccgacatgctgctgataactccatgctaatgtgaaataattaacataatagccataattaaaagcacgctaacaatgccataaatttatcacacaattttactagctttctgcccctaactgctctctcatcgttaattaaacgtgttgccttttacagaatggatgtttatatatttccaatataaataaattcgaaaccatcctctctctcttcctctttctctcctcctttccttttggtctctcgccatttacaggcacgccttggcgtggaccctgagtggcagacatcttgaaaataaatgaagttttgagatgcaaatccaaacaagaacattaaaatagcctctttttttccaccccgaaaagatccggagaggtatacaagggggtagtggtgggtaagagagttgaaaatcccccgctttgggaaatggaagtaatctgggtgggttggggccttgggtaccacctctgccctttcccaccttccttggtggcggccatccagacaaagaggccggtaatagtttaacaaatctatgaagattttcaagaagcagcagactttgattgttgcgggcgcgggggtgttggggagaaaggaggggaatttttctaatagtcccacccacgttttgctccctcttggacaaagagtaactactcttggtgggggacgcgcccttcactccgcggaacctggtcccaactccccgtattgtaagaaaagtgcacccgcgcgcgggcatgatgattctatctcacatcgcgccaacgacttattcaagccactggcactgtctctgacttaaaagaggagaaaagaggcatatgggttcacttgggcctggtgaggggtaggtgggcaattcccgccttccgcactctaaccgtgcccctcctccagtgttgaccacctaagaacccaaaatgagctgtaattaatttccctttctccatcataaatttttctatccatttcttcccccccatccccccactggacgcacacactaaatctcccctcccctggagacgtctcaatttccttcctatcgatccggactccattcttcttgcctcctgttgctagaacctagatccccactccccgcacccctcattcccaccgcgtccaggtggctttcccagcggggtaccatgtactctgcccgctccagaggaaccgaaggggtttcattccattctcctttggttgaaacatttcaaacatttgagcaggtgaggcagctggctgccatcttcctttttaaatctctcctgggaagttcgcttgttgagactcaaagagtcactcaaactcataattgcgtgtgtgtgtctactcattctccctctatctctccaataaccctttgagactcagaaactttttatccacatacaccctttatcacattttcttccccccactacatgtgtctcactttctctctgtatctgtctcgcttcttccgtctctgtcctacagcttggcggtaactgacgacctgtgagcttttagctgcaaactgcaactacgcggcaaacaatttatttagcccgacatctagccggtctccggcaggaccctgcaccgcgtcgggatcggacccttccgctggggcggcctcctgcgtcaaggccagcaggaaccttcctgtcgccctccccggccgccgcttcgcctccttcccgcccccggaggttgtgcaggcgctatggtccgcctggagggagaaagccggcggccggttcctgagccgagagcggccgcggaaaaatcctctgcctccgctggaaatcgatattaggccggcgcgggcgcgggacgtcggggccgcagccagtaggttgtgcacgtctcatcatttagctaatcgagtcgaaaagtttctgtaagggccggacccagcatcagatggtaacactgattgaacaagagattagcacaatagatctctaaccgaggggaagcgttgcttttcacgctacgcgccgtaattaatggtatgaatcaattaatttgacttttattgtgtcgaaggaaaaaagcgcaacaaatggaaccggcagctgggagttgttcgtcctccacccccttccccagggaggttccaaggagacaccggggaatggacggatcaggctgggccgtggcagagggagggtaggaggcagcgaccagcagcgtggagggagtccagagagctagcctctgcggacggcggaatcgaaattaggctcatttggagactacttcgagaccggtgaggggagccctgtagccaccatcctccggcgcgcatccacacatactagtccacgcgggcccagccaccaaggccgcggcagggccagcgctgcgccccgggcccctgcctttagggctgggcaacccaagcagagcaaaggaggttcctgaatgtgtaaatttccgctttttagctttttttttttttttttttggaccttccgacacttcggttgctgaggcagttgcagacgcgacctctgcagtcctgggcgatggccagccagctcagctcgggtcggtttcgcggaaagctgtctagacggcattgtaaacggttcggagcctgcgggccacaaagctgtggagctacggaaatcaactctgagatgcgttttagggccgtgtgcaacctcgggatcatttagataaagaaaaactgtggaggttggcgggcgtctcaggatagtgtcaccaccccctaccctgctcccagcctcagatgagtagtgttatatcctgggaaactgtctaatggggatgaaagtcaatctgtgtgtctcaatgcctgtaatgaagcaagtttacagatttttaaatttttatttttattttattgaattatttttggtgtgtctaggccaaggaaagaggagatcgtgggtggggaaacagactgagggaatcagaagcaccactgtccatccggaattaaatccacatcccagcatcttctgcaaatatttcactaattatttcctctcggaactcctcccctcgtgctccttcctctggtgaggccggcgctcccctcccaggccgcagcggacagacagggattgggttccgtgtgcctgccacaccaggcaggctcttgcggctcccaactaggcggcctaaatgagggaggaaagaggaggcgcatcgctgattcaccgcgtcaagagcactgactttccttggaggtgtgaggtccacgcaccccagccacgcacttgggggtcggtttgcggtgcctccccctccagtcccagtgaaatccccacagtttttcctactatcactgacttgccttgcactccgcgtgcattggccacacatcctcgcctcctccacccgctccgccgccggttttcttggaagttaaatcttggaggatttgtccacaccttaagagaagaaaatccacgttagctggcagcaacggagatcccagcatgctggcatgcccaagtctgcccaggttcccccaaggccatgcccgccgcccgggaagtcactgcccgcacccctcacgtttcttcagccgcccctgggcgctgcgtctaacctgaagacaccaggcctcttcccggatccactcgacttacccaggccgctgccaatcccagctccttccccagcgcctcatttccgattttttcatatgctaagtcgtttaacaactccaagtagccagttatggcttctttatttataggttccctgctattttacgtcgtttttatttctctcggcaactattctagtagattaatcaatagccattttctgaccttcgggaaccccagctgatgctttttgtggccgcacgaaaaaatacatacaggaaaacacgcccgcatcaagccgggaaagagcaggtaggacctgagtggtttggttgggggagggggaaaaagacatctcagcaggtgtcttccccggaatgagcactgaggccagaggggaatctgaaatctaattagcaggagggagccgggtgcgctgctcttactctttaaagctaaaaacaatgaaacaaaaagcaaaacagagactaagttttgctttttaaaacacgatatgggaacctcgttctaggtcgcccagtccctgtctaaggagtgtgacaaagtgggggggagaagggcggaagggagagggggcggggaaggcagggcagcgacagtcgcacagtcccgcggacgctcccaggcccacgccctgactcgctcacacccacccacactcacacccacccgctccctgggccccagggcccggatccagcctgggtgggggggtctccgggcgggccgcagcgccctccgtgccccggggatgctggcgcacagtgcggagcggagttgcgcgtctctcgtccctttgttgacaattccctgaaccaacttgagtttggccggctcggccgcggccctgacgtcacgcacggtcacgtggccccgcctcccgctggatctttaagtagaaagtaatctatcaggccagtccttaaaacgggactttcgactaccggggcttcggcgtccctgacacccagccccctgcccccccgctactgtccctgcccgcgccctcccgagctgctcggcgcccggcgtcccgcgcccgcctggaccgctcctgcgccccacgccagggccagaggccgaggaaggcgggctaagtgagggggcgcggcgtggagaaccgccggggccgggagcggtagcgagcgcctagtaccgagcgccagggacggcaggagttcgcggagcgcggccgctgggggcggacggcagagcccgcgccacgcgatgcggggccgccgagtgtgagctgagcccagcgggccccaagccacctgcggccccctcccctctccctgccccccatctttcgggggcactcaaaccctcttcccctgagctccgtggcagcccccgaacaccctcatcgcccgctgccccctccccgccgccgctaccaaccccgaggagggatgaccctctccggcggcggcagcgccagcgacatgtccggccagacggtgctgacggccgaggacgtggacatcgatgtggtgggcgagggcgacgacgggctggaagagaaggacagcgacgcaggttgcgatagccccgcggggccgccggagctgcgcctggacgaggcggacgaggtgcccccggcggcaccccatcacggacagcctcagccgccccaccagcagcccctgacattgcccaaggaggcggccggagccggggccggaccggggggcgacgtgggcgcgccggaggcggacggctgcaagggcggtgttggcggcgaggagggcggcgcgagcggcggcgggcctggcgcgggcagcggttcggcgggaggcctggccccgagcaagcccaagaacagcctagtgaagccgccttactcgtacatcgcgctcatcaccatggccatcctgcagagcccgcagaagaagctgaccctgagcggcatctgcgagttcatcagcaaccgcttcccctactacagggagaagttccccgcctggcagaacagcatccgccacaacctctcactcaacgactgcttcgtcaagatcccccgcgagccgggcaacccgggcaagggcaactactggaccctggacccgcagtccgaggacatgttcgacaacggcagcttcctgcggcgccggaaacgcttcaagcgccaccagcaggagcacctgcgcgagcagacggcgctcatgatgcagagcttcggcgcttacagcctggcggcggcggccggcgccgcgggaccctacggccgcccctacggcctgcaccctgcggcggcggccggtgcctattcgcacccggcagcggcggcggccgcggctgctgcggcggcgctccagtacccgtacgcgctgccgccggtggcaccggtgctgcctcccgctgtgccgctgctgccctcgggcgagctgggccgcaaagcggccgccttcggctcacagctcggcccgggcctgcagctgcagctcaatagcctgggcgccgccgcggccgctgcgggcacagcgggcgccgcgggcaccaccgcgtcgctcatcaagtccgagccaagcgcgcggccgtcgttcagcatcgagaacatcataggtgggggccccgcggctcctgggggctcggcggtgggcgctggggtcgccggcggcactgggggttcagggggcggcagcacggcgcagtcgtttctgcggccacccgggaccgtgcagtcggcagcgctcatggccacccaccaaccgctgtcgctgagccggacgactgccaccatcgcgcccattcttagcgtgccactctccggacagtttctgcagcccgcagcctcggccgccgccgctgctgcggccgccgctcaagccaaatggccggcgcaatagggacgcgccaatggccgggacccagggtccggcggcggcctcgagcaacaaatgcacctccaggctgcgcgccctgtcccaagcccggtcccggtcccgctgcccaatcctggactctgcctctccccaatttcctttcccctgagcccccaacgcctaccttccgcggcctccatcccctcgcgcacacctaagctggtcgagcaaactcaccgcgcgcccgccggggatagctttccatacaggtaaaaccgaaaaccgaattttccaaaaatgcaccccgacggcgcctgctcttagtaccg

SEQ ID NO: 13 - DNA, 495 bp, Homo sapiens
  source 1..495: mol_type = genomic DNA
ccgcgccctggaccatccgggcgtagtcccggcagcaaggccttctttccttgctagcctgggcctgccgcagacagaccccagagggagccgcgcccagcccgctgggcggccccggcttcccgcgaccccctccagaccctgggcagaaagagcgccctgctgtcccgacagagccactgtgcttttgagggatcctgacacctagtggctcccgctcccttctccgaagagcaccgggtcctatctgagcattcccgcgactcccagcccctgatcgcagctaagacacccattcgcgcacccggcttctcccacatcctcgtcccaggggttcagctgacactggtagtcgcctgagctgtactctttggggcccaggcgccttggcgggagctcaccctccctgtctccccagctgaccctgccgcgcccccttcatctccgcacgctcccacccggccccctccacaggctgtccagccccgcccctcg

SEQ ID NO: 14 - DNA, 1192 bp, Homo sapiens
  source 1..1192: mol_type = genomic DNA
tcgggcctccgctcgacggactgccttgtccactctccgcctgggaacgggggttcgtgggagcgccttagtggaagtttgtggagctcgggaggtggcatgcacaggcgcctcggagcgcggccccgaggggcgccggcaggcgagaggcctgcactaaccggccgtaagcacagctcttttgtactctgttttccccctaaagacatctgatgcccccagtgaagaaaagccaacagcagcaaagcctgatggagagcatgcagcccgggaagcccagtgactgggagctggagggcaggaagcacgagcggcccgagagccttctggcaccgacgcagttctgcgcggccgagcaggacgtgaaggcgctggccgggcccctgcaggccatcccggagatggacttcgagtcctctccggcggagccgctgggcaacgtggagcgctccctgcgcgccccggccgagctcctgcccgatgcccgcggcttcgtgcccgcggcctacgaagagttcgagtacggcggcgagatcttcgcgctgcccgcgccctacgacgaggagccgttccaggctccggccctcttcgagaactgctcgcctgcctcctccgagtccagcctggacatctgcttcctgcggcccgtcagcttcgccatggaggccgagcggccggagcacccgctgcagccgctgcccaagagcgctacgtcgccggcgggcagcagcagcgcctacaaactggaggcggcggcgcaggcgcacggcaaggccaagccgctgagccgctctctcaaagagttcccgcgtgcgccgccagccgacggcgtggccccacgcctctacagcacgcgcagcagcagcggcggccgcgcgcccatcaaggccgagcgcgccgcgcaggcgcacggcccggccgccgccgccgtcgccgcccgcggcgcatccaggaccttcttcccccaacagaggtcccaaagcgaaaaacagacctatttggaagtaaggagggtaaagtaaaaccgaaccgaaacccacagcgtcgacggccccaggcctagatctgcaggaagcatcccgagttctcctagcgtggagaggagcggggccgggccaggctagggggcggctgcgcgagccgtcggcgggtggaggcggagggagagcaggggcagcccccgcgccctgcg

SEQ ID NO: 15 - DNA, 1001 bp, Homo sapiens
  source 1..1001: mol_type = genomic DNA
cctgggaagagctgctgggtggggctgtggctgccagagtctttcccaaactagcacagaacctgttttgcaaccctggcagggtggaggcaggatccaggccaagagctggtcagcagctgaccccgcccctgcctgacccctgccccttccactgccgaagagcccctggcaaatagtgtaactcagatcgtagagggtgcagattgctagaactcagttccagaaggtttctccacgataatgtcatgacttaagtacacagtttttccatttttgtttcgtaacttgattttttaaagcagtcgctacagaacagaatctagacctgtattttatagcatagctgcttgcatgtatttttcaagacttttctttccctcagagtgatgtttgggttttgtttttttcctgggaagttggtgggggtgggagctacatagcccacctctttccccagtaagattctggtccctaggaagaggggaaaacagctcgggcggctctgaagaggaaatctcaggccctagatgctacaggtcattgttagcaaccccagccgctcccaggaaaccagccagcagcagcggagggcagggctgggcgggcacagggtcccgactatacccagtttgcagttcggcccacccccagcaccaggaatgcccctcccaggctatcgctcctctgcaggcttccgcagctccccagcccctgtgctcctggagcctgcctgcctcctgcccgcctgcgtgactcactgagggccccctccctatctttcactttcacccagcacccagaaggggagtaatttcctcctccatttccttcctcagctcctgggccttgaagagagtaagagaccctcctcgtgtgcagcctttgtcttttcatatatgaagctggagggagggagaggcacagagactaggagggcatccaagtcaccctcacccccagcaagaggggagtggggggatttggacaagaagtgcaga

SEQ ID NO: 16 - DNA, 2001 bp, Homo sapiens
  source 1..2001: mol_type = other DNA
taaatgagtgaatgaatgaaaattattttatttttatttgagctttggttctgccatttgctagcagtgtgactcaagagaagccagtaacccccctgagcttccctagttcacaaaatgcttgtcatgaagtcgacagcttccggaggctgcgaggctcgcaagaaatgcccacatgaatgtgcgcttagggcgtgagtgctcactccagaaaactccaacacagtgaaaaggcagaagcggtgtttttcttttttacatttttataagaatatataaaaaatgatataaatggacatttacggtagtgggggaaggcatatatctacgttaaaaggcaggacatttttaaaagctctattttctaaatgaaaactacgaaagcggggtgggttgtggcgggggcagttgtggccctgtaggaccttcggtgactgatgatctaagtttcccgaggtttctcagagcctctctggttctttcaatcggggatgtctgcagagggcagaaagaaaacaggcgttagaaacctgaggtcaaagatgtgtggcacatcccgccctcctctcttgccgtccctaccggcattgaaatacttatggataaagttctcgcaatggcttcacgtgcatgtacccgccgccaccgctctcccacacctccctggtccagcagctagtccactgcccgcctggctgctccaggcgcgccgaccgctcaagcgctccaggtccacccggcggagggcagagaaagcgcgaccgcgcggcccgcagggttgcaagaagaaaacgagtgttatataatgagtctcagtggttgctcacaatgccaggcgcgaaggcgtgaagatgtggcctttcccttcccgcatccccaggcatcttttgcacctggtgcggagtgagccagccagcttgcgataaccaaagggcgcctcaggctctggcgctcctcggcggaatcccgtagcttccctacgcatgcctgcttctacaaacccacaaatggtttccgatcatttctgaaacaaaatggatgctcatttattcatgtgctctggcttctgccttcctctctaatctcgttgcgtatgggctccagctcgccgttcggttctcccgaggcagcatttacacttgagagtctcaagattattttattcctgagggagcatttgcacttgaaagtctctttttacgtttattcctgaggcagcatttgcacttgagtttctttctcccgtagcttgcattagattctccgaccactctttagcttctcctcctattcacacttcatatttacccattgcattggttttataaactcgctctctgaaaatagattgttatcttccttaacgtctgtttcccaggtcgggcaagatagcttgggactgtaatcccagtactttaggaggaggaggggggatgatcgcttgagcccagataacatggtgagaccttcgtctctattaaacaaacaaacaaacccaggcgtcgtggcgtgcacctgtggtcccagctagtcgggaggctcaggtgggagaaccccttgagccagggagtttgaggctgcagtgagctgtgatcgcgccactgcactccaggttgggcaacagatcgactctgtctccaaatgtaaaccccatgagggcaagactcttgtttggtctcattcaccttggcgtgcccaccacctagaacagggctgatcacgcagtagaatctaaccatataattaattgtgcttgaagagggggtgttggggagtaagagaaggaagggaggagggaagaaatgaaagacttgtgtgtttggattaaatatattaggtttggttaagagtcgttcagtttattcatttgcttgtggcccaattcagtagttttactccctctcccacttggctcctcaggctttttgctcagccctggaaccgcgctgtaattggcagctccttctaaatcgggacccggatgctagctgtaactggagc

SEQ ID NO: 17 - DNA, 1834 bp, Homo sapiens
  source 1..1834: mol_type = other DNA
tcgctccggaatggggaagcggctgcgccctggacggagaggggcggggacttcgcgactgcaggcggagggagggcgggtgtcgctggcgcaggcggtgacagggagacaccgccgccactgagtattcctatgcaagtttcttcatcttcctgtgcatcagtgtttacactggggtaatgataaatgctgtgttgaaaaattatttgatggggccatggaaggaacggaaggaacggcgtcctggcccgctcggggcccgcgcacgccgccaccaagccgcgggggcgggtcggaggggagagttgcgtcagccaggccgctgtcagatgacgagcccggggcgtgacggggtggagcatccccaaaaaagtgcatgcctaggatcccgcccagtgtatccctgcgcgcggcgggccgggctgggcagctttataaacagccgtggtgtgagcctcgaagggaaccatcagcgcctcctgtccacggagctccaggtctacaatggcagcggccgccagccccgcgttccttctgtgcctcccgcttctgcacctgctgtctggctggtcccgggcaggatgggtcggtgagttcggggatgtagcctaagcagggcgggggccaaacctgggaggttgtggactgcagcgggtttcagaggaggggaggcttctggaaggaccggcgcgatctccctgaacgaacatcgcggtctccccgaacgtcgcggtccctccgaacgtcgcggtctccccgaacatcgcggtgcccccgaacatcgctgtctccccgaacatcgcgatctccccgaacatcgtgatctccccagacatgcccagctgaaggcactcagttcccctcggtggctcctttccgccgggtccgcttcctgcggctgctgcttgcccctcaggccaggaggtttctggaaggaccggtgctgtctccccgaacatcgtggtctccccgaacatcgcggcctctccgaacatcgccctctctccgagcaacgcgatctccccgaacatcgcggtctccccgaaaatcgcgatctccccgaacattgccatctcaccgaacatcgcgatctcgccgaacatgcccggctgaaggcactcagttcccctccgcggctcctttccgccgggtctgattcctgcggctgctgcttgccccgcaggccaggaggcttctggtagcaccggcgcgatgcccccgaacatcgcgttctaccccaacatcgcgatccctccgaacatcgtgatcccccccgaacatcgccgtccccccgagtaacgcggtctccccgaacatcgcggtccccccgaacatcgcggtacccccgaacatcgccgtctccccgtacattgcgatcccccgaaacattgcgatctccccgaacatcgcgatctcgccgaacatgcccggctgaaggcactcagttcccctccgcggctcctttcctccgggtccgcttcctgcggctgctgcttgccccataggccaggaggcttctgggtggaccagcgcgatctccccgaatatcgcggtctacccgaacatcgcggcctccccgaacatcgcggtctccccgaacatcgcgatcccccagaacatcgcggcctccccgaacatcgcggtctccccgaacatcgcgatcccccagaacatcgcggtctacccgaacatcgcggcctccccgaacatcgcggtctccccgaacatcgcgatcccccagaacatcgcggtctccccgaacatcgctgtctccccgaacgtgcctggctgaaggcactcagttcccctccggggctcctttccgccgagtccg

SEQ ID NO: 18 - DNA, 597 bp, Homo sapiens
  source 1..597: mol_type = other DNA
acgagtgcgtgcgcttgatctggtttctgctctctgggaggtgagtggccgtgcggggcggtggcagctggcgacacctgcgggctgttgggcaccagcccggggcgggcgctcgcacctgtcgggcgtgcacaaaggcccggcgcacgctgtgggggcggggcctcccgggttggccaatgaaaagctggcactgggtcggaggcgccagccaagtggggggcggagcttccaccaccggccaatggggatctggcttcgggatgtgggcggggtccacccggtcgcaacccgttgagtctctgcacagctgccgcgctgacgcgttttccgcgtgtcccgagccccggcggccccgcgagctcggtccgtgcggggaaagcagggctgacgccgtctgcggagaggactgcgcagccgggcttgtgtggggccgcgcgtaacggcagcggctactccctgcccaggccggccagcacagggccatggccgaggcggctgcgcctccggtaagggcgaccctcatggaggcttggggacgtggagccgagtcctgaattcgccaggaggatgttccaccccccaccatctccggcg

SEQ ID NO: 19 - DNA, 481 bp, Homo sapiens
  source 1..481: mol_type = other DNA
tcggatcggcctcccacgcgaagcttgctccccaccagcatccccacgttggtggcgacgctgccccggccccacggatacttccgcgcctgtcagactccctgatgaactacccttcccagagtaccgcgggagctcgggctcctgagggcgacggtcctctgatggcagatgcgggagaaactctggcgtcaggcggccctcgcgtggagcacacgaagtcgtggcttattctggcttcagtatgtggggtggagaaggcgatccacgcagctgcgtctatttcctgtggatcaatcgcaaaatacgttctgtaagccccgcccccactgcgtgcgggcggcttttgtctccacggcaaccgtcaactctggaaacgcctgtctttctccatggcaactgtctacgccgcaggctggagctgcccattaccggagcccgtaagcagtatgggtgctggacaaacagcgtgatcgggtcg

SEQ ID NO: 20 - DNA, 1001 bp, Homo sapiens
  source 1..1001: mol_type = other DNA
gtctgtgttccttttcttaactgtaagaagaaggctctggtttcttcaggttataatttcattaaaataattttattgttttctgacctgaaaaaattcagaatatgtatatctgcttgatattttcttttgggcatcttggtgcaacacttaaaatctatttcattttgtagtttgggagccataattgcagcttcaccaggcttggttcttcttggcccgggcccttcccttcccttgctggttagtaccagccgagctggtttgctttttccctttttggtactattctcctcctccttcctccacgttaccttctgccacggcctctcttctttttccctccattttcaatttacacttacattttccctcctcctcctggccctccctagtttttcccctcccctggtttctagctcctttttgctttctgtttgtgttactgagggcagtgctccaattacctcatatttggagagaggaagctgcagccaatccggtttctgtctgcttttaggtcaagtgatttctgaactgcagtgagatgctttgaatttgtcttgttgcagctctgagcctgtaagatggctgtctgaatcggcagcggctggaagagacagagagaggcggggagggagggagaaagaattggagggattgccggcatagtgcatgtttttaaatgtgcatcgaatccgatgaggccaaggttgggatttctgtgggatcccaggactggcttagctgcgtttttgctgagattaggagaggaaggaaatgggaaattcactgggctgttttaaggagccgaaagagtcaatagctattcctgagaaggctcccatatctcctaagaaaagggttcggttcaaaaggaggtggagagggaagaaaatccctactccagaggcatctcaccaggaagaaacctcagaaggaactggagtcattgaagagactgaaaccctaacgaagttaacagagagtctccaaaagga

SEQ ID NO: 21 - DNA, 206 bp, Homo sapiens
  source 1..206: mol_type = other DNA
acgccaccggtcgaggacggcaggagacccccgagtgcagagaaagctcaaaccggcagcgaagtcggtcctagccaagctgaaaaaacgtctcggatttcgcggacagcggcctagacacagcccgatcttccagtcctagtgccctggtcgagacggttctatccttttgcaaagaagccggaaagagctgggtcccgggggcg

SEQ ID NO: 22 - DNA, 2001 bp, Homo sapiens
  source 1..2001: mol_type = other DNA
acccttgtaggccggatgcggtggcttacgcctgtaatcccagaactctgggtggctgaggcgggtggatcacctgaggttgggagttcaagactagcctgaccaacatggagaaaccctgtctctactaaataaatacaaaattagccgggcgtggtggcgcatgcctgtaatcccagctactcgggaggctgaggcaggagaattgcttgaagccgggaggcggaggttgtggtgagccaagctcgcgccattgcactctggcctgggcaacaagagagacactccatctcaaaaaaaaaaaaaaaaaatagaacaacccttctaaatgtaatccacagctcactcaccttagtccacacaatgaccaccacattttggatgtctccattctgaagcactccccagatttccagacctgggtgttcagccacctacttaatgcctacttaatgtctctgaaacatctcaaactcttacatgaccaaataaagctcctgttgtctccagtgaatattactgttaataccaacttctccatctcagttgaagaaccatggggtcatcgctgaatcctgtttcactccctcgctgtctacatcagaaaatttagttgctccctttaaaaatttgcatccagaatgcaacacatctcctaatcaatgactctggtccattaccctggactggctgtagcttccactctgatcttctttcctcttccctcaaccccacagtctgctctccacgctaacgggatggaccctgttaggactttggtaagatcacctccctcttgtaacccaaatctctcattacctccagaataggtacccaacttctcaggcagccactgcagtcctgactccttccccctgctctttgttcccagctaaaaggaaacagatctatggtttcctcaaaaatctcagcttagttttactaagcacttgcgcctcctgataccagtgccagagataacctttcacaagtttccactggctgacaaaaatgggaacacctcagtataacccctgtaacctctggcatggacttaagagccctgggcttggaatttctccagggcaccagacccaggattggggtaacagcacttaagaatactaggaaaccacaatcccaagaacatgggggtagaggctactgagggaccgaacactctccacttccctatgtgagttccatacgcccttctacaactgggagaaccagggaaagaggaatgcatccctggtgaggctagatgagctcaagcctccctgtagccctgcctggccctgaactcaggctggctgttttactttctggtctcagtgctgtcacctcttgccaactgtagggcaatgaaaaaaagatgtagcctcccactatctcaatgtcctcatcgccccatcgctgctcttcctgtgaacagtctttggaaaagtttttaaaccctaacatagggcgggcacggtggctcacgcctgtaatcccagcactttgggaggccgaggcaggaggatcacttgtcaggagttccagaccagtctggccaaaatggtgaaatcccgtctctactaaaaatacaaaaaattagccggacgttgtaatcccagctgcaggcttgtaatcccagctgctggggaggctgaggcaggagaatcgcttgaacccgggagtcggaggttgcagtgacccgagatcgcgtcattgcactccagcctgggcgataagagcgaaactccgtctcaaagaaaaaaaaactaacataaatggcgtccctcctttgttcagaactctccgtggcttctagcatcctcacaatgacagtacaaccctaggagtaactccgcctcatattcttcgttccctgcagaaaacagctttccgaattctcctggctcagtcgcgcctcaacctttgcacgcgccggttcctccgcctgtcacgctctcccacacctcgtcacacgcagtgtcaaaaaaagggccccaccca

SEQ ID NO: 23 - DNA, 561 bp, Homo sapiens
  source 1..561: mol_type = other DNA
tcgcccggctcaaccccgacgtccgcgccccggccgcctgttggccatggcgggcctgggcctgggctccgccgttcccgtgtggctggccgaggacgacctcggctgcatcatctgccaggggctgctggactggcccgccacgctgccctgcggccacagcttctgccgccactgcctggaggccctgtggggcgcccgcgacgcccgccgctgggcctgccccacttgccgccagggcgccgcgcagcagccgcacctgcggaagaacacgctactgcaggacctggccgacaagtaccgccgcgccgcacgcgagatacaggcgggctccgaccctgcccactgcccctgcccgggctccagttccctctccagcgcggccgcgaggccccggcgccgcccggaactgcagcgggtagggaggccgggcccgcagctcccctggctcccccgggctgcccgccgcctgaccctttcccatgtggctcgaacccctttcctcagccgttctacttttacgttccttttctcagtctaaaagtcgagttccgctcttcg

SEQ ID NO: 24 - DNA, 2001 bp, Homo sapiens
  source 1..2001: mol_type = other DNA
gaaagttcctctgttgctctgggagagggcgggggagagcaggctcgagagccaggctcctccgaggctggtcttgaggcacttctctagtagcttctccaaaagactgagagtgccggcgtaggtatgacagtgagggtacctcacagacccttctccaaagtctggcgggccttggggtttttcggggccaccaggctcggtggaatttttgaaacgctttcgaaatacatagtttcctctgtggagtgagtgcctacaacgcgcaggccggactgatcccccgttgctgcaggttggtgccccaagctgcgggtgctcgggcgccaactaaagccagctctgtccagacgcggaaagaaaaatgggctgtgaaaaagcaaaaggcctcgtctttgaatgaaagttaaacattaaaatctgaccctagagttgtctaaagatcgcggaattttgaagctccggcagagcggactaaaaaacggtgctatgagagatggtgagaatactctaggcatgaacgtgtgcgtgtgtgtttgtgtgtgtgtgtgtgtttcattcttcccgcaaaacaattttttgtttttttcctattcccggtttgttatcggcctagggcgggagaaccacgcagcggcttctgggccctaaggacaaaagagttaaaacaatgaggctcacccgggaagagacgctgccctgggcacaatagggtcgcctgcattactcctccatacacacatctttaaatgtgtccctgtgtgtgttcgttagggtgctgtattacagaaaaagaaaggcctaaaaacacccccagccctggtcgcgcctttcgctaccgcctgagtctggagccgacagctccacctcttctgctccctggaccgccgcgtctccacgccacggcgccctttttactaaaagatcttttctcatcctatcagcaaatcgttaagaaaggcttagccattgcgggggctccaacttaaggattcccccggcccactaaaaggctaggcccggcctgtagcccagctccgcagaaagccagagggtgctgggctttcagcttcttcctcctagacacttgccccacaaatatatttcgttttctctaatccaaatacccatctttttcttttttaaaaaatgataacgtaatgggaaatgaccaaccgaactctgttacataaagttagttctgttagatcttccaccccacccccatcccgcgggagcgagtaaatagaattcatgagcttagctccccaggttcacgctctggaatggtttctttttgcctcattccctaagttttctctcttctgcctcctgaatggagctcaggctaaggagaacggcagaaagagcaaactctgatctgaatctctaattatgaccccatgtattacccatttgaacataaggccctagacgggctccgtgcgatctggggcctcccaagagaaaacttccccgggacaggacgtctgccacgcgcagctaaacaacttctgttttttccgccgtggggaaaataaaagaaccttacaaattctaaggcgtcataacccctgcaagaacttctaactgtatgaaggcccacgcgagattttgacaatagataaatgagctgaggaaatagggtctggccagcgaagggaaacacacagtagccctgggtgcctttctggaatgcccacgcaggggtccgcgtggacaagcacttgcattcaaatacaggaaaaggcttggacggtcgaaataaatctccttttaattttcttttcatcgactaataaaaataattccccagcactaaactcaaataccgtaacgggccacaaaaacacggagaattcataaaactctatctctgcaggtcacccgctaatcgcattattattagcctcgggagcatggaaattgaactgtcactgcctaaagagaaaatgtaagcgacagctgtccctcctctgagttggacagctttgtggctga

SEQ ID NO: 25 - DNA, 2001 bp, Homo sapiens
  source 1..2001: mol_type = other DNA
gggcagaaatgaaatcaactgtggcaaggccttggctgctttcacggaggagtttttctgcgccagtgtctttttccttccctttaaaataaaattaaaaatagcaagcacttctcaggcattcatcagagatagatagatgcacgaggattgagtgggcattttcataaagaatgaggccggctgttatagaccggcggcctagcagatgaaaacttaattagcgtgcctgtcctaaaacctaggcataaatctccctctgccttttggataacgctatatctttgcttatgagaaatgggatgtgagcaactcgctgcacatttctctgattctccaggtcttggtcggctgacacgcattcgatcaagtttaaaggaatgcgcataaatcagcaagcccctagcgtctccttgggagaggtccgcaaatccaggagggcgcctctgaacccaccgggtctggggattagcagtccagggcaacctccgtctctgctcctgaactcgggaattcacagaggaagcaagacactgcatcttcaccaaggcctccaaacacatgcagcagagtgcaatctgcacttacatgtattacaaagtgaaatctgtgtcaactctccgcacacaaatgttgcatctgcagctgaatttcactgcctagtggtgaatttttaagaaaagatttcaactaggttgttttaatttttttcttcccttttctgttaattttttttaaaaacccacaacttgaataacttgaatgggtggcttcagctctgcatcagtcacaaataggagtgaaatgcatagcgacatttaacaatcatccacttaaaataagtaaataaatatgatagtactgagagcagatagaaaaagtagcgtttttttttaaagtcccatttttattttcttaattcaggaagagttttctttttagaaaaaaatactttaatcaggctttcaacaacattatccatgggtcagtggctgatactattattcctatttttcaggaggtggctggtctctccttgatttttgtttttgtttttgtttttgttttaaggttttagactgattgctatttgggcattaaaggagccataataaataatccatgcccactttaggttatctggtagatccacagaaattttaaataggaggagagttaggtaagatcgacactatcaatgaccattttagaactggggggaaaaaatccccacaacaaccctgaaatgtcttctgtcattacagtttcaaaaactagagagagaaaaaaagaaggctactactttacccagggttcctgtagtggtgatggctttcgaaaggggcgggatcccggctggagagctgctgttggcctccttcctaggctcgaggctcagaatatttcttacatctaaagaaaaatatcccctgtcaacagaagagtcccttttggagctgttcttaaacacacagtttgatccagctttgaggggattttccaccactttaaacattttgggagaaagttgttactttggcttgatggcagctcatttggaaatggagtactgtttggaacaagaggtggagaggtgggtctgaagcaacattatcatttgtttccacaagtggagtgaaaatcctcagggcagcaaaatataattgaatttctcgagacctttcgatatgtatgtttcaacaccagcctgtttttgagacagctttagagactctttcgtaattctcatctataaagaagttgtgagtcctcaggagaggttggagaggtttccggcagccacttttgtaaccaatcaatattattttccataaaatgatgaatctggttcttccattcactattactttcctctaacgtaaagataaaattagcctgcatctcacaattctgcatcccacggctactgattccaccaacattttaatacatatgcgcatagcatagatttgacaaaaacacattatcctatgtgtatat

SEQ ID NO: 26 - DNA, 516 bp, Homo sapiens
  source 1..516: mol_type = other DNA
gcggcatccgggatctggcgccgcttttgcgtcaggcttctgcctgagctcggttagggcctcaccgacctgcttccacccctcagggaggcctcagtgattcggccacagcctcagcctccgtcgctctgtgacctgcgggtattggatgattcgtagctaagactctacgacatccctgaagccgggaaatggtgagtgtgccgggcagggcgtccggaggcgacgtggcggggaggccttatcggaaccagcgggaaatggcggcagcggtacccagtctgcgaacggagtccccgctgccgccgctcagccctcggtcctcagtcccctccggtgagggacccgcgctcctgtcgggggacccgcgctcctgtcggggtccccgcaaggctgctctggcccagcctgcagccctccttgtgcagttttgcgcccgcagccccgcaccttccccgggctgtggggtgaggagtagctcatctggaagacgcctgcgtcgcgtgcgcgatgccg

SEQ ID NO: 27 - DNA, 329 bp, Homo sapiens
  source 1..329: mol_type = other DNA
acgaacgcctcagtgtccccgaccctgggcagcggggactcgagcaggcgcccctcactgatggctttagaacgtgggtgggggaaggtgtgtgaggacgggaagacgccgcactcacctgagttggcgtcctcagagtggccgctgccatcagactctgcgggtagagctgggccgggagcgacgggcgacattggtagggacccggggacagcggtccctatcccaggcctgacgtgggtcccccagggcggcgtcgccaaggcttagacgctttcgtgcaggagggacgacgactcccctcacgccttcgtggccccaactcggcg

SEQ ID NO: 28 - DNA, 4240 bp, Homo sapiens
  source 1..4240: mol_type = other DNA
ccgcagaaattactcgtgcgcaccatttccgctgtgggggcattcgtacaagtttccgctgcacacacagcctcccgggccctctcctccaaggctctgccggatcttccaacgaaatcccagagcagcctgcgctggggagcccgcaagtctctccagatctctgcaccccgcaccgcccggaatctgggacggcgcccacgcagggctgggccaagggcagagctcgcaccctgccttcacgcccggttcacttgcgtccacgaaagcagcgtgccggcctcctccatcttcccactcgcgcaacgcacggcgacccgcgcgacacttctgcaatctgaaggcttgcttcttacaaataaagggccagagtctcacacttgccttcgttggagggacttagaagatcctccccacgtccacaccttgtaggaaatgcaaaacagatcgatgaaattaaacagttgcatttggaagccccagaaagacctaaagacatcgtgccggtttgttggagagagggttgcgggacagggggagcgggccttacgcaacagaaaaggtgggcacagcgcgctcaaaatgacccagtgaggagttggtgccgccgggccagaggctgcgagtccagctggctctggacttgctccgcaggcgtcagacgccgtgggaacctgtgtctgcttcttctctccaaagtgtatcggttaaaaaaaaataaaagtagtagtagtagtagtggtaaggaaaaaaataaaaataaaaaggagacacaattaaccaggtcataaaagctagggcaccttcgaccagggctctggccctccagcgatcgttttgcgttgtttctcttctcaaaagtagtctcagacccctgcctttccgctgcagctctgcgacttccccaaactccttaatcctgtaaattctgcaagaaactcccatcctgcaagctgcttttccccctcccccctgcgttccttttttctctccccacccgcgccgcctctctatgcccctctcttctcagaaaaattcctgccccccgcgcgccccaaagcccgggctgcaaacttttccccgccgggcgcctctgcgccagatgccggagcgtctccacaaagcctgagcatctgcacaagttcgcagcctaactgcgggataaagacgtttcccccgtagcttaactagaaaagcgccatcgatgggtgtgttaaacgggataactagagatttcaaacaccttttatttgcctgtcttgaaaaaaaaatctaaatgaatacgcccgctaccaaaaggcaaaataaaaccaaccttaagggtttttgttgttttttttttttttcaaaagtggcgatagggactgtttggacctgactccaacctgcgccctcccttcctctatgaccctcctgcgcttttcctggaacccaaagctctgacttcgtcaaacttacacaattaaaggcaggcggaagaacgcgggctgggaagcaagcgggaagattctagaatggaagggagcccgccgagcgccgcgagccgcgccaggccgggtccgatggagcaggcggggattcctcccccaggcggacccccgccaccagccctgccgggagctcgcggcctgcggagcgcccgggctggccgctcaccgcccgcttcccccagcgaacgactcggggaagctccaggaggccatctgtgctgacggttcacaccagacaggaccacttgcaaggacaaaaataagaaatttaggaaacgaaaaaagacgtactggggcgaggggcgcgggcgcggcgacgacggggccgggggcacatcctggcggccgctcggggagagaggacacgcgcgggaaggagcgcggcgggtgcacggccgcgggtgggagtacgcgcctgtgcgcgcggggcgagggcgagggcgcgtgcgtgtgaccgcggggagggggcgggcgcgtgtgcggggagcgcgccgcgccaggggccgagtgtgtggggccgatccagaagtgcgcagccccctcacctggcccccgtgtcatccccgaaatcccgggaaagggtgggccgcgcgcgggagtttggtggagttggaactttcggtcgcgctcgctgcccactccgctggcgcccggtggcccgtggtgaagggggactagggtggggaacaccggggccctgcggtcccctccctttcctgtatttaagaagccgccggcggcgcagaggcccaggcgggctggcgcgggggcgaggcggcccggtggcagcagcgggcggggcgggcgctccggagtcggtggggcccgcgggttggggggcggggagaggggggagtggaagggagggggaacgcaggggagggagaggaggggaggagccgcgcggcccgcgccgcttccgaaccggaaagttggtcttgccgaagtcctgccaccccggcgtgcgcactccgctccgctccggccgcgagcctccgagcccggccggccgccgggggaagcccgcggaggggacgcggggccgggcgagaaggtccggagagcggggggcacctgagcccgggcgggcccgccgcgctgagcggcgctgagagccgcggcggagcagcgaaggcggccggccgaccccgcgcgcccggaacaggaggcgcggcgcccgagcggcccgggcgagacaaaggcgccgggtcggagccctgcccgcggccgctcgctccgggaggggccgcccggcggcggcggcggggggggcgcgggcggcggcgcagacactctataaaggggcgagcccggcgcgccggcggagacggcgccgcgcggacgccgccaaagtttgctgcctgcgccctgcggagggacggccaccgcggcccgcgccgcacccgggccccgccacagccgcacccggggcggccgaggagcgcggcgccggagcccgcgatgtgaggcggcgccgggcagcgcgcgccccggtcccgaggcgccgcggccccctcctcgtcggcgcggccgctaattgcgagcgcggcctcatttgcataggccgccggagtccgctggagcccggccaatcggcgcggccctccgctaatggccatgcattattcaccagcctaattgctcagccccatgcgcggcccgcgcagccgccgccgccccgcgccccgcgccgcgcgcccgccaggccgccccgcgccgtccccgccggccgccccgctgatgccgctgccccgcgcggggcccgagcgccgctagcagcatgtctcggcgcaagcaggccaagccccagcacctcaagtcggacgaggagctgctgccgcctgacggggctcccgagcacggtgagggccggggctgcggggtggccggggggtctggggctgcccgtccgggctggggaagcgcgtgcggcgggagcggatgcgcgcgtccgggagcgggagaaagttccctgcttcctgcgggcaagcgtccgccccgcgccaggccggccgcggggccccgggtacttcgccggagcgcgcgcggccgccgagagagttgtgggcgaagtaaacttggctcctctcctcggagtcggggagctgcccgcgaagggcgccgaggccgcggccggctcgaggacggctcggaggccggggcgggagggagtccacggtgcctccgccgccgcgccgccccccagggtctctgcgccaggacgctgaggccggcggcggcggggaaggcgaccgcagcccacctaccgctggacgcgggttggggaccccgccgcccggccagctttgttcgggggcccgcggcccctcccgggcccccgcaccgcctcgggtgacccgcggtgtcccagcgcgttgacgcagcctgtgatccctcgcgaggcgaggagaaggtcgggggcttggctctgcctaatggccgcccggggaattaagctgggggtgagcgcagcggcggcggcctgggcctggcccctgctcgcggcgtgtttccggggcgttcgttgcagcgtctgcgcgggccttttctctcccgtctttttggatccgccgaggccgggcgctggagacctcggctttgcagtcatttcgctggtaggagcgtcctcttcgaaacatccaagagcaaagggcaggcgccgcgaaagttaagagactggcaaagggctggacttcccagagtggcgccttagccccgcaaagtttggggcgcccccacccccttcgtcg

SEQ ID NO: 29 - DNA, 2188 bp, Homo sapiens
  source 1..2188: mol_type = other DNA
gcgcgcgcggagcccgctgagacttgaatcaatctggtctaacggtttcccctaaaccgctaggagccctcaatcggcgggacagcagggcgcggtgagtcaccgccggtgactaagcgaccccacccctctccctcgggctttcctctgccaccgccgtctcgcaactcccgccgtccgaagctggactgagcccgttaggtccctcgacagaacctcccctccccccaacatctctccgccaaggcaagtcgatggacagaggcgcgggccggagcagcccccctttccaagcgggcggcgcgcgaggctgcggcgaggcctgagccctgcgttcctgcgctgtgcgcgcccccaccccgcgttccaatctcaggcgctctttgtttctttctccgcgacttcagatctgagggattccttactctttcctcttcccgctcctttgcccgcgggtctccccgcctgaccgcagccccgagaccgccgcgcacctcctcccacgcccctttggcgtggtgccaccggacccctctggttcagtcccaggcggacccccccctcaccgcgcgaccccgcctttttcagcaccccagggtgagcccagctcagactatcatccggaaagcccccaaaagtcccagcccagcgctgaagtaacgggaccatgcccagtcccaggccccggagcaggaaggctcgagggcgcccccaccccacccgcccaccctccccgcttctcgctaggtccctattggctggcgcgctccgcggctgggatggcagtgggaggggaccctctttcctaacggggttataaaaacagcgccctcggcggggtccagtcctctgccactctcgctccgaggtccccgcgccagagacgcagccgcgctcccaccacccacacccaccgcgccctcgttcgcctcttctccgggagccagtccgcgccaccgccgccgcccaggccatcgccaccctccgcagccatgtccaccaggtccgtgtcctcgtcctcctaccgcaggatgttcggcggcccgggcaccgcgagccggccgagctccagccggagctacgtgactacgtccacccgcacctacagcctgggcagcgcgctgcgccccagcaccagccgcagcctctacgcctcgtccccgggcggcgtgtatgccacgcgctcctctgccgtgcgcctgcggagcagcgtgcccggggtgcggctcctgcaggactcggtggacttctcgctggccgacgccatcaacaccgagttcaagaacacccgcaccaacgagaaggtggagctgcaggagctgaatgaccgcttcgccaactacatcgacaaggtgcgcttcctggagcagcagaataagatcctgctggccgagctcgagcagctcaagggccaaggcaagtcgcgcctgggggacctctacgaggaggagatgcgggagctgcgccggcaggtggaccagctaaccaacgacaaagcccgcgtcgaggtggagcgcgacaacctggccgaggacatcatgcgcctccgggagaagtaaggctgcgcccatgcaagtagctgggcctcgggagggggctggagggagaggggaacgcccccccggcccccgcgagagctgccacgcccttggggatgtggccggggggaggcctgccagggagacagcggagagcggggctgtggctgtggtggcgcagccccgcccagaacccagaccttgcagttcgcatttcctcctctgtccccacacattgcccaaggacgctccgtttcaagttacagatttcttaaaactaccactttgtgtgcagttgaaggcccttgggcacaatgagagccagtcctccaaactttcagaaagtttcctgccccttctggcaggctgccaatcaccgggcgggagaaggaaggaggggaaggcggtggagggagcgagacaaagggatggtccctcgggggcggggatggcggggctgtcctgtaggtctgtgcggccaccgtgattgcccctctgcgcggtgcccgaagtcccgctgaaacctgccgagggcagcaggtctgaaagctgcaggcgctagttgcgcggaggtggcgcagctgctctggaggcgcagagcgaatacgtggtgtttgggtgtggccgccccgcccctggcggtttcctcg

SEQ ID NO: 30 - DNA, 2933 bp, Homo sapiens
  source 1..2933: mol_type = other DNA
gcgccggtccggagccggagcgcgggaatcactcgctgcctcagcccaagcgggttcactgggtgcctgcggcagctgcgcaggtggagagcgcccagcctgggaggcagtagtacgggtaatagtaggagggctgcagtggcagaagcgagggtggccgcagcacttcgccgggcaggtattgtctctggtcgtcgcgcaccagcacctttacggccaccttcttggcggcgggcgccgaggccagcaggtcggctgccatctgccggcgctttgtcttgtagcgacggttctggaaccagattttcacctgcgtctcggtgagcttcagcgacgcggccaggtctgcgcgctcgggcccggacaggtagcgctggtggttaaagcggcgctccagctcgaagacctgcgcgtgggagaaagcggcccgcgagcgcttcttgcgtggcttgggcgccgccggctcctcctcctcctccgcgacgcctgccggcccgctgccgcccccgccgccggccccgctgcacagcgcggacacgtgtgcacctctggggccaacaccgtcgtcctcggtccttgggctgcggtcgcctgcggaccccggtgggaacagaaacaagagactgtcagcgccacagacgaggtgaggccgggcctcaactgcaggggtcacgggagtggggcggaaatacactttgatcccactcaagcggagcggaggtctgggaggccctgggcccgggagaccagtcttagactcttgccccactgggtatcccatctaggcctcttctggggagggcggcagactcagccgctgtgtcaacgctgtgttgtcgagaccagctccccaccctctctgggccccaggctcccctcagtaacttggggcactcgacccgagcatccgcgaaagccctcccggctctcagcgttgagcattgggattctagactgcatttccgtctctctgcttgggttcacgcgcctctccacacttagttcacacgcacacacgcgcgcgtcctcgcagcacacacttgtctggtgcaggtaagggaaggtggaggcggatcctggggccaaaggtatttagaatctttcaccctcagccgcctgggattgctgtgagagacatggaaacaggctgagccgaggccttagatgagaggatggactggagagtaaagagggagggttgcccctgcatcgagtttttggaccctgatcccacaccagcttctcggtctcgtacccgcccttccgaagaactccagcagaaaggtccagcggtcccctgtgcttgaggcctacagaagcttgtacccaactagggcaggcacccgggtcttccagaccacaggacaggacaggccacggctgaggaggcctctctcctgcctccaggatgaactaaagacccaatccgggatcttcggcctagggctgctctcccagacctggggtctgagaaagccaaaccagccctttccccaaagctctagttctgcagattctcagctctggcccactcggaggtgttcttcaccacctatccacctactgtggggcccggccctgggaccttgaactggcaggtctctggtccagagctaggtcactggctacctgaggtctctgaacccctcacttttccgcttccctgattttggggatttggggacagacacggcagaaagcactggcgacgaactcaaaaactcccgaacgcaaggggcagcggttctcccaacccagtctaatgcacattggcccaggatgtctcaggcctcaccccaggacgtagggctctgaggagctactccggtctctcgcgggctcagttcccgaagtgatagagcagctcgcgccagagcgcagaacttcgggatttggccagcctccgagccccagggcgcagggtgctcaagccgaccaccccactcggcgtggttgccctccgcgtccatcccctcagcccggcccccatccccgcgaagccgcagcagacctgagacgctggcggacatctcgctgtcgctccggcccgcggcttcctcctctaggtctttggaagcggccagctcacagaccggctggccgaggctcaaggatccccccgcaaggccggccccgctggccccccgcgcgtccgcgcagcgccgcctgctctcgttctcctcgctgagcgcggagtccgagtcccagccttccgggctctccgcagtccgccccgcagctgttctggtaccggcaggagacgccagcagagagtcctcggcgccccccaacgcgcccgcgtccctctccccaaagagccgccaacagcagacagcgggagccgcggccaccgatgccgctgtgcccccgggcgccgggcgcccctctggcgcggccagcccgccgcgctcctctttcttgttgaggatcgcctggatggagaaggacgtcaaggtgttggcgccgcgcacagccatctgcgccgcgggcaggagcggccggcggggcgggcagctggggcgccgagcagctccgagcgggacagagagcgccggcggccgcagcgcgagtgagctgggtgtgcgaggccgccgccgcccactgctgcgcggcccagcagctcccgccccactccgtcccaggatcagcgccgaccctcgcccccaccttagaggcccaccccgcccggagaccccctccccccgaatccagagccagacgctctcctttcgcagctcagctggattatctcatcgcttctcgcccttaggggcgggctggggtctgccccctcgggggacgtgaaggaggattggcgggggcccctccgtggcagcagtcccctcccgagcgccgccggggcgcacagcccgagtcactttttctttgcgcgtctgtcccttcctcgcctgcaggatttcgctcctggcccg

SEQ ID NO: 31 - DNA, 2001 bp, Homo sapiens
  source 1..2001: mol_type = other DNA
agtgtcacatcaacaaatttacacatcaatctaccgcagctaacttcgtaacaatgggagaaacattcagaataatactgagcatcctaccaagggtctgaaaaattgaattcaaatactctgtgtgtaaaatgcctagactctgtcattccagcacatctatgatctgatctagcaagtatatcgttagactacaaattacctttttcctatgacgtgtaaaactccattaaaaatgaattcttcctaataaagttttttatggcgtctaaaattgctgtgaatgttacaccttttacaatcaccttttagccagaaagccattatttgtagaatcctcctgtatttcagttatttgtcacctatttaggctgggcctaatagcaaaactgtcccccgttactgaattcagagaattattcgggcacacgatttatttcctatcttgattagactcctgagcccgtgccccagcctctcgctaatctccctggaccagacaactccattagaatctggcacccacgtttgttctgcctaacactgcaggaaggacagagacttcaaagcacgtgtttgtttttttgttttgtttttggctaccaagaagccaaatttctgtatcctctaccattcaaaaccccaattcaacaaatttacacgggggtttttcctccacgttaagcagttagtcgggtactagagatacacatataaaacacagactctgccctcaaacaacccaatgagcagaaaattctcttaggcaccaaaacgctgtaatagattcaagtgtgtagaggagaagtttggtagagtggatatgacgctttctttctttgtagtacagaaaagataaatctgtagaaaagggagaaagacaactgggtagaaaatttatttcaaatatctaacccaaatcttcaacagattttccattttaaatattccaaaaagtgtaccattgtatattatactaaatgcaggttcatttatcacttaaaaatttttaagctaaaaaatctcaaacaattaacatttgggaagaaaaacaggactgatacacaaagtagtcaaaatatttcagctttctaaactgtatgcactggactaactgttcaatattagaatatctctacatttgaatttggatagcccacagtgataaatactggactgaaaaatctgacatcgaacatatgcaaaactaatggctactatgaaaaaagatagaatggggagagaaaacttgaatgtgccaaaacatttaaacgctctttaaaatatcctgagatgctaaattaaggacaaaacgattagagttccaagaatacaaattttcatctctttcaagattcaactgaatattgaatctcattgagattatgaaatattctctaagcatgtgcttaacttctatttggctttccgcatttcaccacagtgaacagcccattctttttccttgtttacaccaaatgctcgttttgaacacaactcaaaatggaattccaggcccaaaagtcaccacccctactttcacccccacaggcagctacttaacagataaggaattcaagtgcaggacctgaaggtcttatttccatgcaaatttcacaatccccgttacttgcccagatacaacaattaaagcttaaaaggtggcgggagtgggggacttgaggactggtctgaggagaaagtgaatctcccaagggttcctaaatggttttgcttccagtataaaaactgcgagctaccagtagaatttaacaacagctcaaccttgcatttggaacagttactatatagttcactttcttttttcatgggggcggggtatggtgtcttacctactcttaaatttgaacgtattaacaggttcccctccgcgcacactgacatatttcttatcccccataatgaattcagccatatggcattctttcccatcgaaggccatcgggaatggctttaggaagctgattttcaagctttaag

SEQ ID NO: 32 - DNA, 567 bp, Homo sapiens
  source 1..567: mol_type = other DNA
tcggcggcccccccgctgtctggcggacacttgttagtggctgcggagaagccactcacaaagtttcccatcccgttgagggaaggggtcctgactgcgccagcggggcaggcccagaaggcgcggtatctgggaggtccggccgccgcagacgaccccgccgaggcccaaagtgcgccagcttctccgcgcccctccgcctcctcctcctcctcctccctgcagaggggcgcacgcgcacagacacacgcacgcacgcacgcacttacacacaaaaggaagtcatggaaggtgctggtccctgcatacaggcacactcgcgcgggacacacacacaccccccaaaaagaggcgtgcggggttcgccagacggtgggcaaaagcccgtcctcccccccttccagggcctgctcacttcagggagcgcccactcgcccagccacgggccaagagcgcacggacccaggcgggcggcagcccacccgccaccacgcagctccacttcgctgttccacagccaccaaccgcacagccggcacagtcccgcccgcgcagctggcccaatcg

SEQ ID NO: 33 - DNA, 1001 bp, Homo sapiens
  source 1..1001: mol_type = other DNA
ggcatagtttaaaactatccctgctcattctttaaaataagtccacagtagagaataagacatcggaaaatacaaacatttcttcatatccgaatctatttgaatcctaagatgcagatacggagagttcagagtgccatcagtacagggcagagaggttgaagagctcaggaacagacatagggtgggggaaaggggtaggggcaacgacgctgacttttggttaacaaagcccttccaggctgcggagcaacctcctctgcccttcacctgcccggcccatctctggccaagaagaccctgccgccaaatccccacacccagtccaggtcgcagtgcacagactggcccttccgaagcccctcagcggtagcccgactccgaagctcaccgaggcatccgtgagaggagatgccacctagcgcagatcacatctgctctgaatccttgacaaccgcagcccaaagaatgataaactacaaaggccggaaatgcgtcaccgcggcccgctctccgcgaaacagcggttccggctgtgttccttctaggaaggccggaggtttccacacctctgtggtcgtcactctgaatcccgtctgtagtcttaagtgagatactaggtgacacattgtcttccacgcggcaatataataacggccaacatagtgttttaacacgtattaattcattaccccgcataacaaccctgtgagttaggtacaattatctccatttaacaggtgaggaaactgaagcacatttctacatttattagttgccatttcctgcaaagaataccctttcttttccctgccgtctcattttatcacgatgaactcatggattcctttacaaataattactgttattattatgttgatgctcaaattatttaaaatttggtcagttggagccctttcacactgctccctctcttttctttttttgacaaagtctccaggctggagtgcagtggatgcgatctcagctcactgcaacct

SEQ ID NO: 34 - DNA, 383 bp, Homo sapiens
  source 1..383: mol_type = other DNA
tcgcacgttcgcaggcgcgggcttcctgtgcgcggccgagcccgggcccagcgccgcctgcagcctcgggaagggagcggatagcggagccccgagccgcccgcagagcaagcgcggggaaccaaggagacgctcctggcactgcaggtacgccgacttcagtctcgcgctcccgcccgcctttcctctcttgaacgtggcagggacgccgggggacttcggtgcgagggtcaccgccgggttaactggcgaggcaaggcgggggcagcgcgcacgtggccgtggagcccggcctggtcccgcgcgcgcctgcgggtgccccctggggactcagtggtgtcgcctcgcccgggaccagagattgcgctggatggattcccgcg

SEQ ID NO: 35 - DNA, 279 bp, Homo sapiens
  source 1..279: mol_type = other DNA
ccgccagggcacggccccccctgcgccccaaactgagcggcaaagtcagggcccgcggccggatgctcagagctaaaggccgcggaggacagatgtgcttcttcctccttcccgcgtctccccatacaagtactaccccgcacgtcccatcaggcttgcctgtgggccaggattcagggtcctgagccgaaacctaccaggagagagaaggctctggagacctctgtaacagtcgtgcggagaagacaaagtcagctgcgtgcgtctcctccggcgccg

SEQ ID NO: 36 - DNA, 2775 bp, Homo sapiens
  source 1..2775: mol_type = other DNA
tcggagtcacgtgagcgccgaggcccctcccgcggcaggcggcgaaagggcttgcgcgccctcccctcctccacagccccccgcccctcgcgggcccgcccctccaggcgaggccaacctccgcgcccgccgcccgagcctcagcggtccgggaggagctcccggcggcgctcggcagagccctcggccggtgccccgcggccgccgcgctcccagggctactggcgcagcgcacggagaacccggttctcggcgcggtgcgtcgtgctgggcccccgcgccgggccacctgaagccagaggatttggggcgcactgaagggactgcgtctcccagctcgaacccggcttaagtggggccgggagcgaggtcgggaaagtctcacccgcccaaagcctcaccaccgagaggcacttaaaaaggaaagcgcagagggaccctgcccacgcgcgtgtacacacacacccccccacacacacacaagcaaacacgagctccccgccacttcctccccagggtctcctcaaggccaaatattgctcccaatgacagccagtcaccccttggcgaacgcctgctaaggctccgaagagccgggccaccgatctagctcccggctgaaagcagccgaccttgtcacgcgcggggccgggaatgggagggagggtgttagagggtgatcgctgtgggaaagtgagagggagcggctgttagtcattgctccgggtccattaccgagaatccccaaacctagtccgccgctgcgtggcccctctccccatgcaaagcagacccccgaagaagccatgccaggctgagggacagacgccggggctcgaagctccgggcagattcagaaagaggcgtcgctgcagaaaggacgcatcacagttttcagatcttaatgtggccgaggttttacaactcccgacccggcgcagaaaggaaatcccaccatgttccccggagtcgagaaaacggtgaacagctttcggcctgcgctcgacctctgcgtctgcgtctctctcgcctcggcttcccttattttttaaaccaccaccacactccttcccccgccacttccttcccccacccccttcctccgttgcaccagcagcagagtcgcacgcagcaaatactccttcaagaattttacctacctacagttcaagcagttactgggatgtcctgactaatcgaagatgctgccgcgcgcgtgggtcgctctgcgcaagggcctcttcgaaaacccgactaggcgcaactcagcgttcagcagggccgggagcgccaggtcgtccccggggcccgggccccatgactcctgccccaaagcccactccacccgacctccctttcctgaggctgttcccagttgctgctttgggtcgctccggagctcaagaactcgggttgcctgccgccccactctccacgcacatacttggttttcttcttaggggcattggcaggtagactttgaggaagaaaagtaaaggatcgaacagctcagccctccctcccgaccgtggatgcccggagtcgaccaacacctcaggtccgggtgcggaggccgcgggcgcccctgcgcgaccgtccgcgcccggcaagagccgcgcggctttcgcctttgctggtcccgcgccaccgctggggcgggctgcgaaagggttgggaagagcaaagggtttttttgttttgttttgagacgcagaagccctttaaaaagcccggcgaggagaggtccagaagtagagaaagcagacggaggcaagctgtgcccgcggggcaaagggacagtagaaggggcgggcgcccgggttccccggaaaaccctcggccccaaggaatctcctggggcgggagagcgcggttctaaaaccgagaggataggaaggggaagggggagttgtgtttcaatttcggattcaccaggattcatctctagtcacatttttcttctcaaatttttaaatcgaaaagataaaagccaaaagaactttcatccccagagctttttattgggggaaaggaatgtaactcggggtggttgtccttcacttccctactcgaatcttctcctaatgccgaaatgtgtttacaggtagcctcagtttaccaagtatgtatcttttgggggtttaacctctcacaaagccttcaactcacaaaccgcgatccttggaaaccatcctccaaagcagtgcttggaggcctctaaggcccccggaccaactcccgctggaagaagcctgcagggactcgggaatcacgggaacctttcccgtcggttccgggcctggagggccaggaagagccgcgcgtccgcctttcgtcccgccaggaactccccataggacacgacaccgcaggaacaagcgtcctgggagcccctgggatcttggctgtcgtctctagggaccctacaccgtgaaatgatagaggcgaggttccttgggttccgcaagtcgacgaaaatagctcgtggagaaggcgcgtcctgcaactgcagttcgcaagctctcagggcgccccgccagctgggggccagattgggtgacactcccctcgacgcagcctccggagcggcgcgcactctccagaggccagcaggactgcgctctctaccgcagaacctgctccagctaggtgttctctccccatctcgccgtcgctctgccccctcactctctctggacctcagagccggttctctccttcctcctcccgcgctttccgtccggggatcgcaacctccagcccgtgggcaacgcg

SEQ ID NO: 37 - DNA, 2255 bp, Homo sapiens
  source 1..2255: mol_type = other DNA
ccgctttagaggcagcgcttatagcgctagctggtcgtggaatgcgattacagcgtctccattggagaccgctgagtgcctcggtttccctgtctgtgcaaagtgcactccccagacgccgctgcctcgagggaccaggaaatgcgtctgggggcgccaggaaagatgagaagataaagtcacgatgcgtccagctagctatagacacaagcagaggagccagtaggccaaaggagacgcacagctgatccgtgccgaggcgcgggctccactccctgaagtggagggacccttgaatctttccttgcgtaggcgcgcggcagagcagcgatttggcgaaaagggccgagactcaggatgcctgcaatgcgagcgaggggcggacagggcgcacggggcgcggcaaggctgcgaggggcgggcctgggccctgagcctcctgcacttccagccacagctctgggccttgggggcgggaaggggtggagccacgtggggaggagcaaaacccggaggtcccgggcaccttgggcagagccagagcggcgggagccggtcctgggcgcgttgccccgggagcgcccgtcgtccgggcagagcgcagccgcaaccgcgaccacagccgcagtcgctttccagcctgccttcggtgcgcagcgggggaacagggctagtgcagccgccggaggggggcacgggctcctctcccatcccagagctactgggctgcccttgctgtcctcgccgccccagcagaccccggccggacctgccacctgcgccctggttgcgccatggatccttcggaaaagaagatatcggtgtggatctgccaggaagagaagctggtgtccggcctctcccgccgcaccacttgctccgacgttgtgcgagtgcttttggaggacggctgccggcggcgacggagacagcggcggagccggcggctggggtcggccggcgacccgcatggcccgggagagctgcccgaacccccgaacgaggacgacgaggacgacgacgaggcgctgccgcagggcatgctgtgcgggcccccgcagtgctattgcatcgtggagaagtggcgcggctttgagcgcatcctccccaacaagacgcgcatcttgcgcctctgggctgcctggggcgaagagcaagagaatgtgcgcttcgtgctagtgcgcagcgaggcatcgctgcctaacgccggcccccgcagcgccgaggcgcgcgtagtgctgagccgagagcgcccctgtccggcccgcggggccccggcgcggcccagcctggccatgacccaggagaaacagcggcgagtggtgcgcaaggcctttcgcaaactggccaagctcaaccggcggcgccagcagcagacaccgtcgtcctgttcgtccacttcgtcgtccactgcctcgtcctgctcttcgtcgccgcggacccacgagagcgcgtcggtggagcgcatggagacgctggtgcatctggtgctttcccaggaccacacaattcgccagcaggtgcagcggctccacgagctggaccgcgagatcgatcactacgaggccaaggtgcacctggaccgcatgcggcgtcacggggtcaactacgtgcaggacacttacttggttggggcaggcatcgagctcgacgggtccagaccgggagaggagccagaagaggtggcggcggaggcggaggaggcggcggcggcgccccctctagccggcgaggcgcaggcggcggcgctggaggagctggcccggcgctgcgacgacttgctgcggcttcaggagcaacgggttcagcaggaggagttgctggagcgcctttcagccgagattcaggaggaactcaaccagaggtggatgcgacggcgccaggaggagctggcggcgcgggaggagcccctggagcccgacggtggccccgacggcgagctgctgctggagcaggaacgggtcaggacgcagctcagtaccagcctttacattgggctgcggctcaacacggacctagaggccgtcaagtcggacttggattacagccagcagcaatgggacagcaagaagcgcgagctacagggccttctgcaaactttgcacactttggagctgacggtggcaccggatggggctcctggctctggcagtccctcgcgggaacctgggcctcaagcctgcgccgacatgtgggtggaccaggcccgtggactggccaagagcggtcctggcaacgacgaagactcggatacg

SEQ ID NO: 38 - DNA, 875 bp, Homo sapiens
  source 1..875: mol_type = other DNA
ccgcgccacccctcggctctctctctctctctccctaccccgcaggatctacaccggctgtgacatggaccgcctgaccccctcgcccaacgactcgccgcgctcgcagatcgtgcccggggcccgctacgccatggccggctctttcctgcaggaccagttcgtgagcaactacgccaaggcccgcttccacccgggcgcgggcgcgggccccgggccgggtacggaccgcagcgtgccgcacaccaacgggctgctgtcgccgcagcaggccgaggacccgggcgcgccctcgccgcaacgctggtttgtgacgccggccaacaaccggctggacttcgcggcctcggcctatgacacggccacggacttcgcgggcaacgcggccacgctgctctcttacgcggcggcgggcgtgaaggcgctgccgctgcaggctgcaggctgcactggccgcccgctcggctactacgccgacccgtcgggctggggcgcccgcagtcccccgcagtactgcggcaccaagtcgggctcggtgctgccctgctggcccaacagcgccgcggccgccgcgcgcatggccggcgccaatccctacctgggcgaggaggccgagggcctggccgccgagcgctcgccgctgccgcccggcgccgccgaggacgccaagcccaaggacctgtccgattccagctggatcgagacgccctcctcgatcaagtccatcgactccagcgactcggggatttacgagcaggccaagcggaggcggatctcgccggccgacacgcccgtgtccgagagttcgtccccgctcaagagcgaggtgctggcccagcgggactgcgagaagaactgcgccaaggacattagcg

SEQ ID NO: 39 - DNA, 975 bp, Homo sapiens
  source 1..975: mol_type = other DNA
ccgccgggtcactggagtctcagccttccggaatccgagccggcccgccccactccccgcccttcgcggtcccgcccacgacctctccccacgcctcccgctccggcccccaacctcccggtcggacgttcgttcccggctctagccggcctccgcgcctctggcctctttccttccggccgtcccgacggagatatttcttcaatactccataaatacaccccgccgcggaacccacccggagtgagacgcccaacacgtcgtcgaactggggttggccgggggccgctccccgccgcgggcccgcagactcgtggcgtcgccccgcagctccgcctggccgacggggaaccggccgagacccggacacgcacgcccgggaggacaaaagcgcgggcggaccccgcaggctgggaccccggcggctggcccgctccccgagaagggccgtggtcggggggctctcactcacgagccgctggctctgggtcagccctgcccccagggcagcgctccatcatgaggctggcggggcgctgagccgtggcgtcctcgctcctgcgctgcccctctgcatcctggccccttccctgcacacgcagagctgccacactgagcgcccctcagcttacttaagctcggcaaggctggagaaggccgtctgggtgaccgggcggagggggatgctggggaaggaagaattcaggcagctgcaaagagcgcgcgaatatattcattcgacatacctcatgggcgcctaccctgggcctggtccggggcgggtgtttgcggggtggggccgaagcaggggcgtcgccgagttgaagacgtgtactccgagcgctcctgcgttcattcattcgctgggtggagagaggaaggacaagagccccgcgccgatcggaggggagcagaatagtaggcacagttagagggtcttcacggtgcgtttcggaaccttggctgcccggctcg

SEQ ID NO: 40 - DNA, 1284 bp, Homo sapiens
  source 1..1284: mol_type = other DNA
tcgacaaacgcaaagcgacccaaaccctggagggtcacatcccggctgctacaaacctcggcggggcggccccgctcttgcggccgggacagcgcagcggcagcaggggccgcaggggacccgcagattggcacgccgctccccatccccgcagcgcgtctgcaccggagactctgcggggattgtagccggagggcgggccgggctccgaggcgctgctcaggcattggggtttgtcctcatgagctccacgtcggcgtgcaccatctccctcaccagctcctgcaacacaggggtgggcgtgagggaggagcttctgccactctctcctggtgacaccccaccccgggtgtcggccccagagaggcctccgcgtccctcgttccagctcccctcacttctcccgcaccccgccttccgggctttgggcatcgcaggcgcctcaggcgcccgaccctgagagctgccgccctgcagcccggggccccgcagcgggcggcgtgcgccctaagagatactcacatcgaaagcgacccggggcttccagttcagcttctgtttcgctttggtgcagtcgccctgcagaaagtcctagggaagaagagggggagacgaagcaggcgtgggtcgtgggggtgggggcagcaggtcccgagccccgggaactcccaccgttccgctccctctgggcgcacaaggctccgggtttccctgctttcggtccctgctgtgcgcgttcagttgcggctctcggcgccgtaaatcactaggtcgcggttaagaatgtgctgtgcggacccgtgaggaccgtgaccgcgatccacccccagctacctccacacctcttctccccaaggcgtcccttgggctcttaatgctttttttttttttttttttttttttttataacatgaagttgtcagggacgctcctatgagaactgtttggaattgctgcacttctctggctaggagggaagtgagtaaatcaccaggcgcccctcccagctgcccgtgtccctgcgccgctcagctcctgccgcagggctggccgcgccaagcgcgcgtcctacccaaagccaccagccccgcggggaagggactcgggctgtggggcgcgaggccccaggactcggggacccctctacctcggcggcagcgtgcgaccctctttctaacgcggccgtggatgtttcttcccgggccgcagccaagcgcggttcttcctgggcggtggctttgggcttttcgtacccacagtcaagtcagttcacgtcgcctcccg

SEQ ID NO: 41 - DNA, 1001 bp, Homo sapiens
  source 1..1001: mol_type = other DNA
actgctctaaatacttcatatatattaactcctctattctgtacttctgttcccgttttatacagcaggaaattgaaacactgagaggttaagtaactaaagttacagagctagagtgacaggagtaaagcttcaactcaggcaacccagacttccagagttctgatctccactactaagctgctagcatagcttttctggtaactatttttaattcaaatataattcgagtgatctatctaacaagtcatcactctgacaactcagtgacttgtaatgtaaaattattcattgtaattcatttaatattattgtttctctgtgctgcaaaaatcatagcaatcgagatgtaatttattactctccctcccacctccggcatcttgtgctaatccttctgccctgcggacctcccccgactctttactatgcgtgtcaactgccatcaacttccttgcttgctggggactggggccgcgagggcatacccccgaggggtacggggctagggctaggcaggctgtgcggttgggcggggccctgtgccccactgcggagtgcgggtcgggaagcggagagagaagcagctgtgtaatccgctggatgcggaccagggcgctccccattcccgtcgggagcccgccgattggctgggtgtgggcgcacgtgaccgacatgtggctgtattggtgcagcccgccagggtgtcactggagacagaatggaggtgctgccggactcggaaatggggtaggtgctggagccaccatggccaggcttgctgcggggggaggggggaaggtggttttccctcgcactgtcttaaaccgatggcctttccttggcacagggtccactgcagcatgccaaacgaggaggcaggggcgtcgtccccccgccccccactgcagcactggagatggatttcctgtacttcggatccagggtttttgacagaagaggaagaagggggaggggtagaagtgttaaggggagtctgc

SEQ ID NO: 42 - DNA, 859 bp, Homo sapiens
  source 1..859: mol_type = other DNA
acgcagaggccgtggcatctggccgcagctgggctgcagtgcgtgcgcgcctggcctggtggtccgatgggaagcccggggcggggcagccgcggggcgggggcggggcgtcgcggagataggccacgcccctgcccgcccgcgcaggcgcgctgcgggtcgttagctgtcagagccaagcggcgggctggcggcgggctccgacgtctgcgccaggacctggctggctgagcccggcgcagcagcagcagccagggcagcgcggcccctactccctgtcaggtcgtagaggcgagcagggaccagctggtcgccggcccctcgggcaagatggggaaccgggagatggaggagctgatcccgctggtgaaccgtctgcaggacgcgttttcggcgctgggacagagctgcctgctggagctgccgcagatcgccgtggtgggcggccagagcgccggcaagagctcggtgctcgagaacttcgtgggcaggtaagcgcgcagggcgcggagtaaggatgcggcagtggggcgaccccgctgcgggccgttggaacgtggacgggcagcgggagccagagggtggatggaccaggcgctgcggtggaatggggggcagagtggaatggggggcagagtggcggtgtccgtggggcgggcggggtcctccagctctgggcatcctccgtcccctgccaccccccgcctggtggccctcctgcctgcctttcatcgtgcgatacaaagccatttcctccctgtcctccagtcggggagtcgggggaggggtccgccccgggctcgacccccaccccctcggtgcgcgccagccccgggcagcctccctgcgtagcgcgccg

SEQ ID NO: 43 - DNA, 2001 bp, Homo sapiens
  source 1..2001: mol_type = other DNA
gacagaaaacagccagagcgcaccactcacctgagtgccaggtaaacacctgggcgcgacagggacaggaaacaagggtagggtgcggaggctggggaggaagaggttggaaaggggggaaataaatgggcggggcctagcaggtcctgtgcggggcttagggccggggcggggcccaggaagactcagcagcgggtgggtgagggtctaaaggcggcaattccgggccgggtgcggtggctcacgcctgtaatcccagcactttggtaggccgaggcgggcggatcacctgagatcaagagctcgagaccagcctgggcaacgtggtgaaaccccgtctctactaaaaatacaaaaattagctgggcgtggtggcgggcgcctgtagtcccagctacttgggaggctgaggcaggagaatcgcttgaacccgggacgtggaggttgcagtgagctgagatcgcgccactgtactccagcctgggtcacaacagggaaactccgtctcaaaaaagaaaaaaaaaaaaggcaattccgagcccagacaaaccttaaggaggggatcctggatcttcagttaagtgggcgacacctggagtgaggggcggggcatatgcagagtaggtgcggcctacaagccaaaaaggagaaagagttggaatggtgggcctggcttatgcgggtgggcggggagagggtggatcctagaggaggtgaggcctaacattgggcgaagaaggcgggagcctgggccaatgagctgacggtaggccggggagggggcggtggggtggggtgggcaatgggcaatgagacggagggcggggccgggacctaatatggcgggtcaggagggtctggaagacgaagaagagggacaggcaatgccaggtctaggactaggagggaggcgcgggcggtattagcggctggaggaggcttcgggaggcccggccgacggccgccgcctggtgctacccacccaggggcgcgcgaccctcccttcggtctggctccaaagacctagcagcactgacttcacccagctgtggttccaacggcgggtccagcggcctcggcccggcgccgtcctcctgctggcccaacaggcccgccagcccgcccctgtacgtctgtgattggacggcggcggccactgatgttcaagcgacaggtcctggcccgggagccaatctgcaggtgttgaggcccaggctccgagagcgggccgaggaggcgtggataccctgattcctagggggcaggcctggttcccccgaggaggacccggcctatgaatgactggagttctggggttctggccgaaagaggaagtgggacagggccgggtgtgatggggcctagagtcacagagccttgcggccctgctgtccctgcaagaagccagcttctggccaggcgcggtggctcacgcctgtaatcccagcactttgggaggccgaggcgggcggatcacgaggtcaggagatcgagaccatcctaacatggtgaaaccctgtctctactaaaaatacaaaaaattagccaggcgtggtggcgggcgcctgtagtcccagctactagggaggctgaggcaggagaacggcgtgaacccaggaggcggaggttgcagtgagctgagattgcgccactgcactccagccagggcgacagagcgagactccgtctcaaaaaaaaaaaaaaaagcagccagcttcttcctcctattttgcaaccttctcccgatatccttgaacattttagggacagccatcacttaaccatagagcaaccctattaagtctaagtagcataatcacattcctgtagtatagatcatgaacctgaaattcgaggatgaagtcatttgcctgaagacatacatcttgtaaaatagccatccgcaaagatgtagggaaaaaggcagcgatctgtggctacacctccccttcctcccggaagcagccactggaacgtttttagctttttctttttttttca

SEQ ID NO: 44 - DNA, 1007 bp, Homo sapiens
  source 1..1007: mol_type = other DNA
acgcggtgaccttgaccccggcccaggccctgctaatgaagaggaaagcccgtacgcactcggcctgacccacggcgaccctctgtgaccaatcatactaccaacctcttaaacagagctccaccgacgcaatgcccaggcataaaaaggccaggccggagagaccgccaccagtcacggaccctggacccagcgcacccgcaccatggccggccccagcctcgcttgctgtctgctcggcctcctggcgctgacctccgcctgctacatccagaactgccccctgggaggcaagagggccgcgccggacctcgacgtgcgcaaggtgagtccccagccctggtcccgcggcgctccggggagggagggacccgcagccacaggggcgcgccccgctccggcctcgcctgagaactccaggagctgagcggattttgacgccccgcccttgaccgcggtcgaggcccccacggcgccccagcgcgtctcagccccgctgtcccgcccgaactccgaaccccggaccccagcatccttgcccggcgcaccccggccggcctcgcagggtcctccgagcgagtccccagcgccgccccggctcccgctcaccccgcccgtccccgcagtgcctcccctgcggccccgggggcaaaggccgctgcttcgggcccaatatctgctgcgcggaagagctgggctgcttcgtgggcaccgccgaagcgctgcgctgccaggaggagaactacctgccgtcgccctgccagtccggccagaaggcgtgcgggagcgggggccgctgcgcggtcttgggcctctgctgcagcccgggtgagcggggcaaggcgctccggggccagggggaggcgggcgggggtgcggccgggattcccctgactccacctcttcctccagacggctgccacgccgaccctgcctgcgacgcggaagccaccttctcccagcgctgaaacttgatggctccgaacaccctcgaagcgcgccactcg